European Patent Specification EP 3 346 826 B1, published February 19, 2025. Title: REDUCTION OF ASPARAGINE CONTENT IN PLANTS. Applicant: Philip Morris Products S.A. The sequence listing filed with the application follows.

SEQUENCE LISTING (24 sequences)

SEQ ID NO: 1 - DNA, 3646 bp, Nicotiana tabacum
atgtgcgggatcttggctgttttgggttgttctgatgattctcaggccaaaagggttcgtgttctcgagctctctcgcaggtaaattatatttcccttcttttctgtattgttaatgttattgtgttgcgttattatattgattctttttatgagaaagtagtttcctgaacgtttgcattttagaataaaagaagactaaagcttaagatagattatatatttagatattcttgacgtggacctatatcttagattcacaatataattttctcggaccaactgttttagcatgacttgtaaatgatgttgatatgaaaagctgtgatttaattagtaggagtaattcatttccatgttacaattacttatctttctcctccttgtgttcttgccactgctagaggcagatctataattcctacttagagtattgaacacattgtacttttgaaattgtaagtgtgcagtttaatatttgttaaaattttgaaggtttttttaattacatgtatatcgtgacgttatatagcctctctacccgcataaggtaggggtaatgtctgcgtacaaataggctgatttcactctgtgttcagttgaatcaatatatgcggcatccaccactgtttgcaaatgcatgggaatggaaaagtcatgcctcatcactgtcacacatgatttttatttatttatttattatatatgattctttaaatctattagtgggtactgaatcttgctaactgatcgattgatgaaacaggttgaagcatcgtggaccagattggagtgggctgtatcaacatggggactgttacttggcacatcagcgtctagctattgttgatcctgcttccggtgatcaacctctgtttaacgaagataagacgattgttgttacggtgggtgcttttaatttcatgtttactctcatttcttgctcagtttactgatgaaaacgaaactaatgctgataactatcaaccaatcaaccacatacaagtaggggtcgactatatgattcattatatcctttcctctattcaaatagttgatgattaatttcatgccaaaaatttcaggtaaatggagagatctacaatcacgagcaacttcgtaagcaaatgcctaatcataagttccggactggcagtgactgtgatgtcattgcacacctagtgagtactcatcttccaacttaggaaacatgtatgtatatgtaaaattattccctgattatattatgtacattaatcagtatgaagaacatggagaagattttgtggacatgctggatgggatcttcgcttttgtgttattggatactcgagataacagctttcttgttgctcgtgatgccattggaattacttccctttatattggttggggacttgatggtaagattccatatgattttctcacttagattttgttattgcaaatgaatatgttgaatccttatatgtactaattgttgtaattctgttccttctcagggtctgtatggatatcatctgagcttaagggcttgaatgatgactgcgaacattttgaagttttcccaccagggcacttgtactctagcaagaatggcggctttaggaggtggtacaatcctccttggttctctgaggccattccttccactcgttatgatcccttagttctcaggcgtgcctttgaaaatgtgagttaatattgttgttgttgaaatggatccaacatgttggttttaaggctatatatcattttgcaggctgttatcaaaaggttgatgactgatgtcccctttggtgttctcctctccgggggactcgattcatccttggttgcttcgattactgctcgctacttggctggtacaaaggctgccaagcagtggggagcacagcttcattccttctgtgttggccttgaggtcagataatcttgagacttgtgtgattacaacattaataacgacaacacctcattcacaagctagtaaggtcagctatatgaaatctgataccgatttgcttgctttcaccgaacagggctcaccggatctcaaggctgcaagagaagttgctgactacttgggaaccgttcaccacgagtttcacttcaccgttcaggttttgatggagcaactctattttcacttgatctatcatcctcttcgtttctcctttgtttacctgatggcaaatgacatgtgttgtatttgcaggatggaattgatgcaattgaagatgttatttaccatattgagacatacgatgtaacgacaatcagagcaagcactcctatgttccttatgtcgcgtaagattaagtcactaggagtgaagatggtcatatctggggaaggatctgatgaagtgtttggtggctacttgtactttcacaaggctcccaacaaggaagagttccacaaggaaacatgtcgcaaggtataagaaagtgcttccagttcctagtttaaataggacaaggagttgagaaaatgttgattttttccctatgcagattaaagcgcttcaccaatatgactgcttaagagcaaataagtcaacatctgcatggggtttagaagctagagtccctttcctagataaggagttcatcaatgttgccatgagtattgatccagagtggaagttggtaagtagttgacccccaattgttgatcgaataaacaatcaactgtccctaaaactatgtatttattcatttcagattaaaccagagcaaaggaggattgaaaagtgggctctaaggagggcctttgatgatgaggagcatccttatctcccaaaggtgtactaaatcgccattttcaaactgatttgcaaatgattttgaatgttatattattaatcaaactaacaatttactcattacattccttgcagcacatcctgtataggcaaaaagaacaattcagtgatggcgtgggctatagttggatagatggactcaaagcacatgctgaacaacatgtgcgtttcaatgactaatcaacgactttctactgctcttatttatcttccaatgcttgtttgttttaaagctgaccgaggaaacaaattttttcctttaataggtgaccaataggatgatgtttaatgcttcacatatattccctcataacacacccattacaaaggaagcatactactataggatgattttcgagcgctttttcccacaggtaatttgttcagataatagtgagaatttatgataaatggactaatttacgtttgttgtcgattttgcaaccttccaacagtgtgagcaagctcacataatcggaattttttgttcaaataataatgcattggaaatcataatgctaaattgagatttacttttaaccatgttcctctaccatttttggttctgcagaattcagctgggctaaccgttcctggaggagcaagtgtggcgtgtagcacagctaaagctgtagagtgggatgcttcttggtcaaagaaccttgatccttcaggcagggctgctattggtgtacataactcggcttatgagaatcatgtacctgctatggctaatgggaatttgaccaaaaaaatcattggtcgtgtgccttctatggtagaagttggtgctgctcccgagctcacaataaagagttag

SEQ ID NO: 2 - protein, 590 aa, Nicotiana tabacum
MCGILAVLGCSDDSQAKRVRVLELSRRLKHRGPDWSGLYQHGDCYLAHQRLAIVDPASGDQPLFNEDKTIVVTVNGEIYNHEQLRKQMPNHKFRTGSDCDVIAHLYEEHGEDFVDMLDGIFAFVLLDTRDNSFLVARDAIGITSLYIGWGLDGSVWISSELKGLNDDCEHFEVFPPGHLYSSKNGGFRRWYNPPWFSEAIPSTRYDPLVLRRAFENAVIKRLMTDVPFGVLLSGGLDSSLVASITARYLAGTKAAKQWGAQLHSFCVGLEGSPDLKAAREVADYLGTVHHEFHFTVQDGIDAIEDVIYHIETYDVTTIRASTPMFLMSRKIKSLGVKMVISGEGSDEVFGGYLYFHKAPNKEEFHKETCRKIKALHQYDCLRANKSTSAWGLEARVPFLDKEFINVAMSIDPEWKLIKPEQRRIEKWALRRAFDDEEHPYLPKHILYRQKEQFSDGVGYSWIDGLKAHAEQHVTNRMMFNASHIFPHNTPITKEAYYYRMIFERFFPQNSAGLTVPGGASVACSTAKAVEWDASWSKNLDPSGRAAIGVHNSAYENHVPAMANGNLTKKIIGRVPSMVEVGAAPELTIKS

SEQ ID NO: 3 - DNA, 4564 bp, Nicotiana tabacum
  misc_feature (3137)..(3137): n is a, c, g, or t
atgtgcgggatcttggctgttttgggttgttctgatgattctcaggccaaaagggttcgtgttctcgagctctctcgcaggtaaattatattcccttcttttctctattgttaatgttattgtgttgcatgcgttattaattctttttatgagaaagtagtttcctgagcgtttggagctgctactgattgcttgcattttagaataaaacttaagatggattatatatttagatattcttgacgtggacctatatcttagattcacaattttctcggaccaactgttttagcatgacttgtatatgatgttgatatgaaaagctgtggtttagtaattcatttccatgttacaattactaatctttctcctatctgtgttcttgccactgctagaggcagatctataattcgtaattagagtattgaacacattgtacttttcaaaattataagtgcgcaatttaatatttgttaaaattttgaaggcttttttaattacatgtatatcgtgtctcgtatagcctctctacccatgtaaggtctgcgtacacattacccgccccatgccctcccgtgaaattttactggggtttgctgttgttgttggtatcgtgtgtcgcatatactttgttctgttgaatcaatatatgcgtcatctgccactgtttgcaaatgcatggaatggaaaagtcatgcctcatcactgtcacacaggatttttatttatttatttatttattatatatgattctttttcttgatgtgaaatctattagtgggtactgaatctggctaactgactaatgaaacaggttgaagcatcgtggaccagattggagtgggctgtatcaacatggggactgttacttggcacatcagcgtctagctattgttgatcctgcttccggtgatcaacctctgtttaacgaagataagacgattgttgttacggtgggtgcttttaatttcatgtttactctcatttcttgctcagtttactgatgaacatgaaactaatgactatcaatcagccaatcaaccacgcttaattccatacaagtaggggtcgactatatgattcattatatcctttcctctattccggttcctttttattcaaatagttgatgattaatttcatgccaaaaatttcaggtaaatggagagatctacaatcacgagcaacttcgcaagcaaatgcctgatcataagttccggactggaagtgactgtgatgtcattgcacacctagtgagtaatctagattactcatcttccaacttaggaaacatgtatgtattcccctgattatttcatcatctttatgtacattaatcagtatgaagaacatggagaagattttgtggacatgctggatgggatcttcgcttttgtgttactggatactcgagataacagctttcttgttgctcgtgatgccattggaattacttccctttatattggttggggacttgatggtaagattccatattattttctcacttagattttgttattgcaaatgaatatgttgaatctttatatgtagtaactgttgtaatttggttccttctcagggtctgtatggatatcatctgagcttaagggcttgaatgatgactgcgaacattttgaagttttcccaccaggacacttgtactctagcaagaatggcggctttaggaggtggtacaatcctctttggttctctgaggctattccttccactccttatgatcccttagttctcaggcgcgcctttgaaaatgtgagttattattgttgttgttgaaatggatccaacatgttggttctaaggctggatatcattgtgcaggctgttatcaaaaggttgatgactgatgtcccttttggtgttctgctctccgggggactcgattcatccttggttgcttcgattactgcccgctacttggctggcacaaaggctgccaagcagtggggagcacagcttcattccttctgtgttggccttgaggtcagataatcttgagatttctgtgattacaacattaataacgaccacacctcattcacaagctagtaaggtcagctatatgaatctgataccgatttgcttgctttcaaacgaacagggatcaccggatctcaaggctgcaagagaagttgctgactacttgggaaccgttcaccacgagtttcacttcaccgttcaggtattgatggagcaactctattttgacttgatctatcatcctctgcgttcccttttgtttacctgatggcaaatgacatgtgtcgtatttgcaggatggaattgatgcaattgaagatgttatttaccatattgagacatacgatgtaacgacaatcagagcaagcactcctatgttccttatgtcgcgtaagattaagtcactaggagtgaagatggttatatctggggaaggctctgatgaagtgtttggtggctacttgtactttcacaaggctcccaacaaggaagagttccacaaggaaacatgtcgcaaggtataaaaaagtgtttccagttccttgtttaaaaccttatttaaataggataagcaacaacaacaacaacaacccagtataatcccactagtggggtctgaggagggtattgtgtatgcagaccttacccctaccctggggtagagaggctgtttcagatagaaactcgactccctccctccaaaaaccttatttaaataggacaaggagttgagaaaatgttgatctttttcctccatctctatgcagattaaagcacttcaccaatatgactgtttaagagcaaataagtcaacatctgcatggggcttagaagctagagtgcctttcctagataaggagttcatcaatgttgccatgagtattgatccagagtggaagttggtaagtagttgaaccccaattgttgatcgaataaacgatcaactgtccctaaaaccttgtattctatccatttcagattaaaccagagcaaaggaggattgagaagtgggctctaaggagggcctttgatgatgaggagcatccctatctcccaaaggtggtactaaatcgcccttttcaaactgatttgcaagtgatttcgaatgttatattgttaaccaaactaacaatttnaaggctctgatgaagtgtttggtggctacttgtactttcacaaggctcccaacaaagaagagttccacaaggaaacatgtcgcaaggtataaaaaagtgtttccagttccttgtttaaaaccttatttaaataggataagcaacaacaacaacaacaacccagtataatcccactagtggggtctgaggagggtattgtgtatgcagaccttacccctaccctggggtagagaggctgtttcagatagaaactcgactccctccctccaaaaaccttatttaaataggacaaggagttgagaaaatgttgatctttttcctccatctctatgcagattaaagcacttcaccaatatgactgtttaagagcaaataagtcaacatctgcatggggcttagaagctagagtgcctttcctagataaggagttcatcaatgttgccatgagtattgatccagagtggaagttggtaagtagttgaaccccaattgttgatcgaataaacgatcaactgtccctaaaaccttgtattctatccatttcagattaaaccagagcaaaggaggattgagaagtgggctctaaggagggcctttgatgatgaggagcatccctatctcccaaaggtggtactaaatcgcccttttcaaactgatttgcaagtgatttcgaatgttatattgttaaccaaactaacaatttactcattacatttcctgcagcacatcctatacaggcagaaagaacaattcagtgatggcgtaggctatagttggatagatggactcaaagcacatgctgaacaacatgtgcgtttcaatgactaatcaacaactttctaatgttcttatttatcttccaatgtttgtttgttttaaagctgacttggaatttttttgtttcctttaataggtgaccaataggatgatgcttaatgcttcacatatattccctcataacacaccgattacaaaggaagcatactattataggatgattttcgagcgctttttcccacaggtaatttgttcatgtattgtgaggattcatgataaattagctaacttatgctggttttcaaccttgcaaccttccgataagtcacattgttggagtttgttgttcaaatgcgagatttacttttaaccatgttcctctggtatttttggttctgcagaattcagctgggctaaccgttcctggaggagcgagtgtggcgtgtagcacagctaaagctgtagagtgggatgcttcttggtcaaagaaccttgatccttcaggaagggctgctattggtgtacataactcagcttatgagaatcatgaacctgctatggctaatgggaatttggccacaaaaatcattggccgtgcgccgtctatggtagaagttggtgctgctcatgagctcacaataaggagttag

SEQ ID NO: 4 - protein, 590 aa, Nicotiana tabacum
MCGILAVLGCSDDSQAKRVRVLELSRRLKHRGPDWSGLYQHGDCYLAHQRLAIVDPASGDQPLFNEDKTIVVTVNGEIYNHEQLRKQMPDHKFRTGSDCDVIAHLYEEHGEDFVDMLDGIFAFVLLDTRDNSFLVARDAIGITSLYIGWGLDGSVWISSELKGLNDDCEHFEVFPPGHLYSSKNGGFRRWYNPLWFSEAIPSTPYDPLVLRRAFENAVIKRLMTDVPFGVLLSGGLDSSLVASITARYLAGTKAAKQWGAQLHSFCVGLEGSPDLKAAREVADYLGTVHHEFHFTVQDGIDAIEDVIYHIETYDVTTIRASTPMFLMSRKIKSLGVKMVISGEGSDEVFGGYLYFHKAPNKEEFHKETCRKIKALHQYDCLRANKSTSAWGLEARVPFLDKEFINVAMSIDPEWKLIKPEQRRIEKWALRRAFDDEEHPYLPKHILYRQKEQFSDGVGYSWIDGLKAHAEQHVTNRMMLNASHIFPHNTPITKEAYYYRMIFERFFPQNSAGLTVPGGASVACSTAKAVEWDASWSKNLDPSGRAAIGVHNSAYENHEPAMANGNLATKIIGRAPSMVEVGAAHELTIRS

SEQ ID NO: 5 - DNA, 5276 bp, Nicotiana tabacum
atgtgtggaatcttggctttgttgggttgttcagatgattctcaggccaaaagggttcgagttcttgagctctctcgcaggcaatttcccctttcttttctcttttattttattactccatcatataattattctactttcaccttttttgttttttaatttcgatttgtttgctttttgctttcttcatttaatgttcttgcattgctctagctcctatacgaataataggagctaaagtaatagagtgaaggattattttggagcaacggtaaagttatttttgtatagttcacaggttggagccgtaaaagcagttactagtgtttgcattagggtaagttgtctatcaggaaagatatttgtagcaattgaccaccctttggcaaaaaattatgcgtaaaatattactacttgttattgattcaaaaaatatgactttgaacatccttgtatagcctagtggcaaagggtgttcaaaatttttgaacacctttattgaattttctggtttcgtcgttgctgtctacaacacactctcgaagtgcggccttccctcaaaccctacgtgaatatggaacgcctagtgtgccgggatgccctttaggctgagtaatagagtactatgttgatatacctaaaatacggaactggcacgagagataaattcagaatttatagcttaattatttaaaatttatcatttgatttatttcaaccagagttcattctagtagagtttatgttgcatatttgtctgatttgcaccatttgttttaatgttcttgcattactctaatttatttatgaataataagctaaactaattgagtttatgttgatgtaactgacctgagttggcagtgatgtttggctacttgaatttaaaacaagattaagacttgtgagttggcagtaattgtttggatacttgaatttagaacaagaataaaacaagattaattaaggatacattattcctaacccggaccctaattctatagattgattattaaatttttcttggaccaaccgtcaccgtgacctgttcatgatggtgatggcaaaagccataatacacttgatttctgttttcaatttttaaggttcttattattatacttattatatactttgaaaattatgggtcaaaattttaatatttgttattccttccgtatgtttgactcaacttggagttcatgaaaaaaaaaaaaaatttttttaaacttgtggtcttaaacaagtcatcgatatatgtgtggttgtgaatcgcctcgttaggataaagtagaaattttaaagttaaactatttcgaaataaaaaagtatgatagtgtttttgggacatactaaaaaggaaataacacataaaatggaacaaagaagtatattttagtgatttttcacatatatatcagtattttgtatcaaaaatgctggttcagttgaactcattgaactgggtgctccatccacctccgagtactgcaacatgtgaccggtggcagatgcaacccttacgtaccagggtcatctgaacctagtataaatatatttgtgaaaaatccctaaaatttcaataattagtagatttaaaaccttaattttaaaactacaatgagttcagttttaaaatctttatatgtcaaacctatcaagattaaatcctggatccaccttttgcatgtgacagtacaatagccttttgtaattgaaacaaatatttgaattttggtaactatttgatcacataggttgaagcatcgtggaccagattggagtgggatatatcaacatggtgatttttacttagcacatcaacgtttagcaattatcgatcctgcttctggtgatcagcctctgtttaatcaagataagacgattgttgttacagtgagtgcctctaatttacctcttttttttttctttttttttttacgatcgcgttgtttagattatttatggatgaaaatttgtatatttgattattgattgtgtgctaaattttgcaggtcaatggagagatttacaatcatgagaaacttcgtaatcttatgcctaatcacaagttcagaactggaagtgattgtgatgttattgcacatcttgtgagttagtttacttttctcattgaccaacttaggccagtgaattatattaggaatttcgggtgtttggatatggtcaaattagcttataagcacttattatcaattttaacatttttatccatacacgtaactgttcattcataaagtcattttagcacttgatgctcatcaacctatgttgttgggactcttcgaaaatgtcagcccgatagcatttcggagagtccgagcaacatagcaatcaactacttttaatcagttaaacgaacatgctcatagtgataacctctggaaaatatgttatagtaaattagaaaaatttatacgatgtctcactatcggtatgtattgatcagtatgaagaatatggagaaaattttgtggacatgttggatggggtgttctcttttgtattgttggatacgcgcgataacagctttcttgctgctcgtgatgcaattggaattactcccctatatattggttggggacttgatggtaagattttctatacaattttccagttagaaattaaaactgaagctattcctatttactattgaagaatcttgatacatgttatttggtatttcgtcgtgttgttatgtctcaggctctgtgtggatttcatctgagctaaaaggattaaatggtgactgtgaacattttgaagttttccctcccggtcacttgtactcgagcaagaatggcgggtttaggagatggtacaatcctcaatggttctctgaggctattccatcaaatccttacgaccccttagttttgagacgtgccttcgaaaatgtgaggcttgttaatgaatctagtgtacaatcttggatgtttttctctcgactttggttttagcactcaaaaagttgtctgtacaaacgatcttggctataaggagtggtggttaattttgcaggctgttatcaaacgattgatgaccgatgtcccctttggtgttctgctctccgggggacttgattcgtctttggttgcttctgtcactgctcgctacttggctggaacaaaagctgctaagcaatggggagcacagcttcattccttctgtgttggtctcgaggtcagactatcaatcctgagcggagacatatttggggcgggttctgtgggttcaactgaacccattgcttttggttcgaaccatatatacaaatccaagaaaatataagatgtgtacatataatatgacactcattctgagcctactgacgctagatactggactcgcctttggtcttgagactttataatagaaaatagatattcaataccaatttctgtttttcttttctgactgacagggctcaccagatctcaaggctgcaagagaagttgctgactatttgggaaccgttcaccacgagttcaccttcacagttcaggtttgtaaatcgtgttgctactccgatttattcatgtgagtctcttctgttttcctcctagaaagcaacaagtgttcatgttttgcaggatggaattgatgctattgaagatgttatttaccatatcgagacatacgatgtaacaacgatcagagcaagcactcctatgttccttatgtcgcgtaagattaaatcactgggagttaagatggtcatatcaggggaaggctcagatgaactgtttggcggctatttgtacttccacaaggctccgaacaaggaagaattccatgtggagacatgtcacaaggtaataaaacacgtcggctcccttggcaagtctgattctccttgtcattgtttgtctcgggttggaataaattgctataattcgagaagaaatgttaatcctgctctttcactcgcatgcagataaaagcgcttcaccaatacgactgtttgagagcaaataaggcaacatcagcatggggcttagaagctagagtaccatttctggataaagagttcatcaacgttgctatgagtatcgatcctgaatggaagatggtaacaaaactgagctccaattgtcaatgagatgagaagcataactgaatatgcacgttctctaaaacttgtttttcatccgtttcagattaaacacgatcatggtaggatcgagaagtgggttcttaggaaggcttttgatgatgaggagcaaccctatctcccaaaggtccacaaagtcatgtttttcctactgatttgccgattagtatggatcaaaactaacatgttttgttcttttatgtactctgcagcatattctgtaccggcagaaagaacaattcagtgatggcgtaggctatagttggatcgatggactcaaagcacatgctgaacaacatgtgagcttctaaataaatccagaactattacatcgttatcgtccaattttcgtttgttttgctgtcagctgatcttggaaacaattcttttctctcaggtgactgataggatgatgcttaatgctgcacatatcttccctcacaacactccaactacaaaggaagcatactattacaggatgattttcgagaggttcttcccacaggtacttatagcgcgagactagaatcatatatctcttaaatggaaacatgaaaaataaaggaggtgttttttctccttggaaaaagtatttactactgattaaagcaccttcattcacccatcttgctacttcgcgtactttactaagttgtggttctaaaaaagaagatttagcttggtatattccatcacgaggaagccacaaaaagattctacttataagaagttggatacttttaatggtgtgagaccttttgggaaaaaccatgcgggcttggcccaaagccgacaatatcacaccatgttaagagtatctttgcttcgttttagccaaacagtacaataagtcaatttttaaaccatgttgttactattgttggatttgcagaattcagcaaggctaactgttcctggaggaccgagtatagcttgcagcacagctaaagctattgagtgggatgcttcgtggtcgaacaaccttgatccttccggtagggctgcaatcggtgtacataactcggcttatgacgatcatctccccgatgttggtaatgggaatttggacacaacgatcatcgataatgtgccgaggatggtaggagtgggtgctgctgcagagctcacaataaggagctag

SEQ ID NO: 6 - protein, 590 aa, Nicotiana tabacum
MCGILALLGCSDDSQAKRVRVLELSRRLKHRGPDWSGIYQHGDFYLAHQRLAIIDPASGDQPLFNQDKTIVVTVNGEIYNHEKLRNLMPNHKFRTGSDCDVIAHLYEEYGENFVDMLDGVFSFVLLDTRDNSFLAARDAIGITPLYIGWGLDGSVWISSELKGLNGDCEHFEVFPPGHLYSSKNGGFRRWYNPQWFSEAIPSNPYDPLVLRRAFENAVIKRLMTDVPFGVLLSGGLDSSLVASVTARYLAGTKAAKQWGAQLHSFCVGLEGSPDLKAAREVADYLGTVHHEFTFTVQDGIDAIEDVIYHIETYDVTTIRASTPMFLMSRKIKSLGVKMVISGEGSDELFGGYLYFHKAPNKEEFHVETCHKIKALHQYDCLRANKATSAWGLEARVPFLDKEFINVAMSIDPEWKMIKHDHGRIEKWVLRKAFDDEEQPYLPKHILYRQKEQFSDGVGYSWIDGLKAHAEQHVTDRMMLNAAHIFPHNTPTTKEAYYYRMIFERFFPQNSARLTVPGGPSIACSTAKAIEWDASWSNNLDPSGRAAIGVHNSAYDDHLPDVGNGNLDTTIIDNVPRMVGVGAAAELTIRS

SEQ ID NO: 7 - DNA, 5926 bp, Nicotiana tabacum
atgacgtagtttagcttgttcgtccacggcataaaaacgcctataaattcggtggtcattttggttcatttacagaatcccacgatcatcttttgtgtattatcattttgccttctttacgtgttcttctctcccaaaatcctgcaaatctttaactatcttcccatatttctctccctctttctctttctttttgttatctactttactacttctattagtagagctttatccaattaaagtcatctatattggatatagtttttactactactttatcttgtttgggaaagaaaagaataaaaaattagagtgtctatattaagtataaaaaggtgaaaaataaaaaagtagtgatcaatcatgtgtgggatcttggctttgttgggttgtccagatgattctcaagccaaaagggttcgagttcttgagctctctcgcaggcaattcccctttcttttctcttttattttattactccatcatattattcaactataatttcaccttttttgtttttcaattaatatttgtctgcttttgctttcttcatttaatgttcttgcattgctctagttcctttatgaataataggctaaagtaatagagtgaaggagtagagtcggagcaacggtgaagctgtctttacatgatctatagctcacgggttcaccatagaagcagccaatggcgaagctagaaaattcaataagggtgttctttcctttgccagtgggctatgcaagggtgttcaaagtctatttttaatcaataacaagtaatattttatcttatagtgaaagcaaccactaatacttgcatttaggtaattagctgtctatcaagggaagttatgtgtggtaagtagtggcggagccagaattttcgttaaggggtgtcaaaatatataaaagtaaacataccaggaaattaaggggagtcaatacatagtatatatacatataatttatttttttacctagctatacagtatattttttccgcgaagtgacaccccttcctataaggtggctccgccactggtggtaagggtggtcaattgaacacccttcgccgaaaaattatactctggatggtgtaaaatattactacttgttactgattcaataaataaattttgaaaacccttgcatagtctagtagcaaagagtgttcaaaattttgaacacatttattgaattctctggtttcgccactgctgtctacatcacatcccttaaggtgcgatcttttttcgaatcatgtgtgaatacgggatgccttgtgttccaggctgcccctttaggctaaagtaatagagtacgtcttaattcttatgttgatcatatacctgaaactcggaactggcacgagagatataaattcagaatttatagcaaatttatcattatgttgcatttgttttaatgttcttgcattactctaatttttttatgaataataagctaaactaattgagtttatgttgatgtaactgacctgagtttggctacttgaaagttaaaacaagattaagacttgtgagttggcagcgattgtttggatacttgaacacgtttaaaacaagattaagacattatgatggatacattattcctaacctgggtgggacctaattctatggattcattattaaaatttcttggacaaaccatcaccatgatctgttcatgatgtttatggcaaaagccataatacactttatttctgtatcacaactactttatacacatgttatagagttttaaaattattttaatatttgttattccttgagtctcctgatatttgactccgcatgaaattcaagaaaaaaaaaagaagatttttaaaatttatagtcgaaaacaagccatcgatatatgtgtggttgttaataacctcgttaggcgtaaagtagaaattttaaagttaaactatttctaaataagaaaatatgatattgtttttgcatagactaataaggaaagtatgacaagtaaaataaaacaaagaagtatattttaatgattttttccgtgtcaaaaatgtcagtttagttgaacttgaactcattgaaactggtgaccagtggtggatgcaaaccttaggtacggaggtcatccgaacctagtatagttatatttgtgaaaaatcactaaaatttcaataattactagatatgaaaccttaattttaaaactacaatgagtgcagttttaaaatctttaaatgtcaaaccgatcaagattaaattatggatccacctttaaatgtcaaaccgacagtacaatagccttttgcaattgaaacaaatataaacattacatttattaaactagttttaattttggttactatttgattacataggttgaagcatcgtggaccagattggagtgggatatatcaacatggtgatttttacttagcacatcaacgtttagcaattatcgatcctacttctggtgatcagcctctgtttaatcaagataagactattgttgttacagtgagtgcctctaatttacccttttttttgtggacgaatgcgttgtttagattactttaattatggctgaaaatttgtatatttgattattgattgtgtgccaaatgttgcaggtcaatggagaaatttacaatcatgagaaacttcgtaatcttatgcctaatcacaagttcagaaccggaagtgattgtgatgttattgcacatcttgtgagttagtttactttactcatcaaccaacttaggctagtgaattcaaaggcggagctagaattttgagtatatgagttctggaatttaggacaagataagttactgggttcggatagattatttagacatattaagtagatttcttaacacaaatacacggcccgagccgaagctattgggttctgccgaacccgtagctagacttgtagctccgccattgagtgaattatataaggaatttcgggtgtttgggtaaacttataagctggtcaaattagcttataagcacttattatcaatttcaacatttctatccaaacacgtaactattcattcgattttagcacttgatgcttatcgactacttttaatcagttaaacgaacaggctcatagtgacaaactctagaaaatatggtattgtaaattagtagaagaatttatacgatgtctcactatcgatatgtattgatcagtatgaagaatatggagaaaattttgtggacatgttggatggggtgttctcttttgtattgttggatacgcgcgataacagctttcttgctgctcgtgatgcgattggaattactcccctctatattggttggggacttgatggtaagattttctatacaattttccaagtagaaattaaaactgaagccattccaatttgctattgtagaatcttgatatatgttatttggtatttcaggctctgtgtggatttcatctgagttaaagggcttaaatgatgattgtgaacattttgaagttttccctcccgggcacttgtactcgagcaagaatggcgggtttaggagatggtacaatcctcaatggttctctgaggctgttccatcaaatccttatgaccccttagttctgaggcgtgccttcgaaaatgtgagaaatgaatctaggaggtttccctctcgactttggacttagcactctaaaaatttgtctgtacaaacgatcttggctataaggagtggttgttaatttcgcaggctgttattaaacggttgatgaccgatgtaccctttggtgttctgctctccgggggacttgattcgtctttggttgcttctgtcactgctcgctacttggctggaacaaaagctgctaagcaatggggagcgcagcttcattccttctgtgttggtctcgaggtcagtcaatcaatcttgagtagaaaaaatttagggtcggttctgtgggtttaacttaactcattgcttttggctcgaaccatatatgcaaatccaaaaagatttaagatgtatacatataatataacactcattctgagcctactgacgctagatactggactgtgcctttggtcttgagacttttgtaatagaaaattgatattcaataccaatttctgttcttttgtgactaacagggctcaccagatctcaaggctgcaagagaagttgctgactatttgggaaccgttcaccacgagttcaccttcacagttcaggtttgtaaatcgcgatgctacttcaatttattcatgtgaggctcttctgttttcctactagaaagcaacatgtgtgcatgttttggcaggacggaattgatgctattgaagatgttatttaccatatcgagacgtatgatgtaacaacgatcagagcaagcacccctatgttccttatgtcgcgtaagattaaatcacttggagtgaagatggtcatatcaggggaaggctcagatgaactgtttggtggctacttgtacttccacaaggctcccaacaaggaagaattccacacggagacatgtcacaaggtaataaaacacatcggcaagtctgattctccttgtcattgtttgtctcgggttggaataaattgctataattcgagatatggaatgagttaagaaatgttaatcatgtttttccattcgcatgcagataaaagcgcttcaccaatacgactgtttgagagcaaataaggcaacatcagcatggggcttagaagctagagtaccatttctggataaagagttcatcaatattgctatgagtatcgatcctgaatggaagatggtaagaaaactgagctccaattgtcaatgagacgagaagcataactgaatatgcgcgttctctaaaacctgtttttcatccgtttcagattaaacacgatcaaggtaggatcgagaagtgggttcttaggaaggcttttgatgatgaggagcacccctatctcccaaaggtccacaaactcatatttttcctactgatttgccaataattatggatcaaaactaacatgtttgttctgttatgtgctctgcagcatattttgtaccggcagaaagaacaattcagcgatggtgtaggctatagttggatcgatgggctcaaagcacatgctgaacaacatgtgagcttccttaataaatccagaactaatgcagcgttatcgtccaatttttgtttgttttactatcaactaattttagtcatgttagtatgtttaccttaggtactatgtttttaaggagtttttagtcgtgtcaagaatttattcgctggtaaaaaatagattgaacttccagtattttctacttttattatgcatatgattggactgagatgaggttaaatggaacaacatggttgaggattaatataaccaattccaacttggttggaattgaggcgtcgtagttgttgttagatctcagaaacaattcttttctctcaggtgactgataggatgatgcttaatgcttcacatatcttccctcacaacactccaactacaaaggaagcatactattacaggatgatttttgagaggttctttccacaggtaatattagtgagagattaaaatctatagattttgtttatggctgaggtttaaatcatagatttcttaagctcaaaaactaaaaccatgtccctgctactgttggatttgcagaattcagcaaggctaactgttcctggaggaccgagtatagcttgcagcacggctaaagctattgagtgggacgcttcttggtcgaacaaccttgatccttccggtagggctgctatcggtgtacataactcagcttatgacgatcatctacccgatgttagtaatgggaatttggacacaacgatcatcgataatgtgccaaggatggtaggagtgggtgcttctgcagagctcacaataaggagctag

SEQ ID NO: 8 - protein, 565 aa, Nicotiana tabacum
MTLKHRGPDWSGIYQHGDFYLAHQRLAIIDPTSGDQPLFNQDKTIVVTVNGEIYNHEKLRNLMPNHKFRTGSDCDVIAHLYEEYGENFVDMLDGVFSFVLLDTRDNSFLAARDAIGITPLYIGWGLDGSVWISSELKGLNDDCEHFEVFPPGHLYSSKNGGFRRWYNPQWFSEAVPSNPYDPLVLRRAFENAVIKRLMTDVPFGVLLSGGLDSSLVASVTARYLAGTKAAKQWGAQLHSFCVGLEGSPDLKAAREVADYLGTVHHEFTFTVQDGIDAIEDVIYHIETYDVTTIRASTPMFLMSRKIKSLGVKMVISGEGSDELFGGYLYFHKAPNKEEFHTETCHKIKALHQYDCLRANKATSAWGLEARVPFLDKEFINIAMSIDPEWKMIKHDQGRIEKWVLRKAFDDEEHPYLPKHILYRQKEQFSDGVGYSWIDGLKAHAEQHVTDRMMLNASHIFPHNTPTTKEAYYYRMIFERFFPQNSARLTVPGGPSIACSTAKAIEWDASWSNNLDPSGRAAIGVHNSAYDDHLPDVSNGNLDTTIIDNVPRMVGVGASAELTIRS

SEQ ID NO: 9 - DNA, 21008 bp, Nicotiana tabacum
  misc_feature (18072)..(18072): n is a, c, g, or t
  misc_feature (19355)..(19462): n is a, c, g, or t
  misc_feature (19541)..(19541): n is a, c, g, or t
  misc_feature (19714)..(19786): n is a, c, g, or t
  misc_feature (20035)..(20035): n is a, c, g, or t
atgtgtggaatactagctgtttttggttgcattgataactctcaggccaagcgttcccgaatcatcgaactttccagaaggtttcttctttttattgctttccgattttctacagcattcttattcttctggggtgtcaatggtatgcatgtgttttggatttgctattcgtgaacttgttcgctttctcgtggtcttcgatttatttttgtcaatttataatcagcgttttttgtatggatttctcttttgaatctctcaaatatatgacatttgatttcctcgagaaaatttggcatttttatggttcttatgatatgtggttaacccctcgctctgcatcgcttcagcgctttaaaacacgaagtgatggctattagtaatactgctagagtggttattgaattacattaaataacgggttgctagtagatcaaattcagaatgacagtgaaatatctctggaaacttgaatccccgttcgattcgctggtaaaacctggctaaaaaatagctttatctcaaaggagagtatgtcactgtgaaattggtggtatgtgttgtttaaggcatgatatgctgctcttaggtgatgtcaagatgataataccatccttttcacactagactcagctttgtagcacttacatctcagttaatcgatggaggaaaatctagtctgctttggggcatattataccaaatgtcttccttttgttttctagtgttgtttctcaagaattgaaaaaccaatctacaatatagtgatataattaactagttaactcttcctgtgttttctgaaaatttccaataattgagaagtgtttactggtcaattagtaaagggagaacggaatatttttttcctctaaagaacttctctttttccatacagaatgactttctatacaaggcctaagtctaatttagtgtctgcgattaagcatcttctgggaacttcacacttgaaagaagtagaactaggagggggcaggtctagaaagataattgcttcagtcatttctcataaaaaacattgcttcagtcattatgtgcattcatatagagttggtcaagctgctaagctgagctaatagtatgatagctgtgactctcgacaaagtaggttgcctcttagggctttatcctttggctccgtaaagaatttctttgggagggctccagagtgggtaggattgttctcatggtaagctgtaacaccaacgaaacaagcctttgtagctgtggaagtccgagggggtggtggtggtggtggtggtgtgagagttagagtggtggaggagaggggaggagtgaagagaagtttatattttaaagaatagggccttgagaacttttagtagtgagcatgcattattattattgttattgttattattattattattattattattattattatattattattattattatattattgttatgtaattacttagctaatgaggtttttccaactgtttccaaattaggaaatgtgttgaaagcatagttaagtatataaaagcgtgttctttctaatatccttagcttttagagcagataatcacaaaatttatcatgataatatagcagacaatttttcctagttcaaatctcatgccacccttcataaaaaatttccacgtgcttggctggcatgttaggggacgtcttggcataattaaacaaatagaattgtccctttctaacagcttaagcttttagatgaggcggtcaacaattcaacaatttgcatttgtttgataagaagatattaaaagaaccttaaaaggtgtcagtatgtgaacaaactcaaggggtagactaactagaagtcaatttaaattttctgcttgtctgtgttttacttcttttgcactatagaaattgcatttccagcattccgaaagctgcttcctttgcatatagacttcacatttccagcgtttctgataagcgttcttgcttattcctgtccttctacttggttgattctcctctcacttagttcactatcttcttgcacgcattttcaaattgttttatcaattctcttgctttcttttcatctgaccccacaaaatacctcccaaaagcctttctgcttttccgagtctgaaattatctgcttattactgcctttcaagtattctgatgcgttgactgtttttttcccttgtagtaatgcatggttcgctgtccaatctctattttgttttttgtgaaccactattctttgttgcttctgtttcgtcatcctcagttccccatcttctcagtttgattttcctcatttaaaaagcgtgtgccccttttcttgtgctaccctctaaaaaatcagttgctgtcatctcgtttgatctgtcatgatcccagttgatgccacatgtttagttctttacctctggacaacttttacttcctgagaaccacgatttcttttcctgaagaaattcttagaaattggttatgtaaaggaaattcccagcaatcaccatttggcctctacctggcttgcttttcaacttaccgacacgtgttcatccccttttaacagatgctgaccattatcttctgcttgttggggcatacttcttacccatggtgttaaccctgatctttcgtatcacatttttcaactcttaattctcacatgtaaagtgcctatctttgcctctttagttgatcttgggttgggctgttaatccaaattctctgggctttgctttgaagtatgataagcggtagctttactacagtaccatattctacattgctacagacgtgaaattatcctgatttgtctttgatgtgatgtctggcaagtgtagattacgccacagaggacctgattggagtggattgcatagccatgatgactgttatcttgctcatcaacggttggcaatagtagacccaacttctggagatcagccactttacaacgaggacaagaccattgttgtcgcggtatggaaatatttattatattttttcttagatattaccggtacatggactttggacaatatttgtgcgttttgatcttctatagtacaaacttttctcgtaggataaatttcctctactttgaatggatcttaacaggaaaatcggaataaacaatttgtgatttcgaaatttttagttcttacatatttggaacatatgcggtaaagtaactaggcgattgactaggtgaatacggagaatttcctctactgttatcaatatttactcagctcatttgaaagatctctgggtcgtctagcagtacagctatttaggcaacttaaccaaatccccttcccatgtgtttcactttcttgacttattttatattttgacattttgcaatgccgaaaataaattgtttttccattttatgacctttaaaatgttgaggtgaagggctaggcggtactttaattgacttatcagcaacaatgtattagatacagagcacaaacttgtttgggtgcctaatttggtattttttgagaacgatggagtaaatggaaatatgaattagcaaaatattgaaatagtagatctgaaaaatgaatgactgaatttagaggaggaccttttcttctttccttgctgaagtggttataagagaattatgtgaagaacatgtaagctttagggtagtgttacaccataacagtcatgctttccctcaactattagtgtagctgatgaatgctttcagaaatgtggctgtttttttgctgcgtattttatgtctttcatcatctcaaaatttattgtgttttaacactgcttggaaggcctagagtcttccgaaaatagtaggttgagaaaacatgagtaagcaaatttcttcctgctggcaattaatcgttttatatgaggtgaagccacacaatctaacatggtcttagacataaaaatattatttttgacatagagcagacagaaatcttgggtctagttgctatctcccttcctaataagatgccctctatcctcattgctatatcccaaaacagattcacactagaatgaataaatctctccttgcagccacatttatattaataagtagtgtaacaccaaaacatttgtgcttctgcaaagtctgttgaagtggacgattaagtaataaattgtgtgagtttgactgaagagaaagtaataaattgggtgagcttctcacatttttcaggataatgtcaattcatctgattgaactttttgaaggacatctccttttctaaaagtttttgttcacttcctgaaaatggttgctttcccaaatttattctcctgtattttccttgtgctttttttttttaccaggatgactctggccttcccttttgcaaatagtgacttcattaccttttaacaaaagaccaaatagcctttgtatgcttgaaatcgaagcagaatttacggctcaatttctctaggagatgtgtagcagtaacataaaacgtggttaaagcaacttgtaagcactgccactgtccaatttgacatgactctattactatttagagtgtcaaatagtgtttcttttgactaccaatttttcaatttcttttttataccttttttctttgactgtgacttatagtatattttatgtagtttcagaatatatattttagtttttaaagaattgatgtctgaaagtacagccaattagatggtttcaccctcgtactttaaatcttataagttgtcttaggttaaaggaataatatgcatgattacattgtttggattgatattcagaagatcaaatgtgccggacaaaagcttgcagaagatataattctgtcattttgttgtttagataaactacccttgtcaaatacctaaaactaattcatacttttcaggatccttcttgattggactactctgatcttcttccatatattgatatcctattctttttgcttttaggttaacggggagatatataaccatagagacttacgggaaaagctgaagtcccaccagtttcgaactggcagtgactgtgaagttattgcacatcttgtaagtactttcagaatatatttagataactatacatgacttctcagtttctgtgcgcagaatgatttcaaaataccatgactcaaatttttcatcaaaagcgaaaaaggtggattgtagtaggagaatgagattttttgtcataatttctttcttatggtacttgaactccgcaatctacctatcgcagtatgaagactatggagaagacttcgttcacatgttggatggaatgttctcctttgtgcttcttgacacccgtgataaaagtttcattgctgctcgggatgcaattggcattacacccctttatatgggatggggtcttgatggtatgtaattgttccatttcataatttttggtatattgtccttttaataaatagcccgtgagctatatgaagttcctttgttgtttccttgttttttatttgactgatgtatctttgttgttttgcctactattaggggtgtcaatggttcggttcggccggttattttataaaatttgtaccataccaatttttaggttattctattatgtataaccaaaattagactttttgaaaccgtcccaatcatgtcggtttctcttcggtatcggtacggttcggttaattttcggtattttttaatatcatgtaaaattcaccagtagaagtagaattgcaataacatacattcttttataggacttagcaaaactctctagatatttttactgtttaaagggtgatgaattaaaaaaaaagaaaagaaagatggctagaatatagatccatcaactattatacaacagcgtaaaagaaatcaaacaaagacaaagaaaatattaatcacacgagttgaaagatataccaaggtaggactcaagaataaagtctatagaagattaaatattcaaaaagataaatctaaattatatgaaaggaaacatattcaattcattgtagtttgctactcataatcgctagaatactttgtgtcttgctaataaagatacttgaaataatttagtttaagtagaagtagcataataggttttatgaattagtattttgagtttaattacttgttggcttgtaataattttcataattccaaggctcaaagaaaatttattgcattattatttttaaacttactaaataaatatattttctacatgtaaaatttattcggtatggttctgtattttttcggtttatttttataaaataaaaaacctaccctaattatcggtgcggttgtagatttatataaaaacctacggtttcttaaaaagaaagctaaaaatcggttcggtgcggtacggttcggtcggtttagtcgattttcgaatatccattgacacccctacctactataatgctggtctcatgctgttgttacaaacaaatgatgtataatagtgcatagtacatgttttcttgccgctgtagatcaacaatgtaccaagaacatctgtcttagctagttcaacctaatcttcagttatctatcattccagtgaataacacatatagagttaggccgacattacctaaggccaactatacaacattgtgaggtgcgactaaggaactctgaacactgatcgggagaaaaagcaacttatccgtgtttgttttgaagtactatgaggaggcagcaaccttgctggatttatcacttgacagtaaatgtcaatggttgaggaacatttttaatgaccggaggagaaacagagaagagaagaaataattgattttaaaaaagcagaatagaaaattttgtgaagtcgtatgttaatttcaatgaagaggatcaacaggtgcaatatttgacttggcacctagcatgtagaagtttctggttggggttgagcatggtaggcactgttgcttttacaactgtcattagagtcggaaacatattgtattcttgagggagcgttgctatggataaaaaaggcctatctactacttgatatttgggcattcagaactagttgtctaggaggaagaaaaggatttaaaatggtgagtattgtaggctttctttgccgtccaggatgcctgggctagttccctgaattgggatactggtggaggatttcctgaaattgatcatggccctgatatgttaggggataagaacattgaaggatcgaaggaaggtgccggcgctaagttttgctagaaatgaacagttccattatggcttttgtcaaagatgggaatggaattggccccaacttctaggcatctccatccatcgtcaggtgaactaaagtaaggttacactggtagaatttttcattatttcatattaagtaaggtgaagccgtcaacaatcattgcgtgagaaggaaccaggaacaaaatctagaagatgtctactaaagtgctaatagataatctgcaaaatttagcacggtaaggctagtgtagatctggttcaaattttaaattggtccaaaatgcgttaataaatgtcgggcctcgttttggtcccccgaaaggttgctaaataaagacttgacaaagaaacaggtgaaggagaagcccaaacatttgaacaaactacacctagcctaaacaaagtgattgtttgcgaggaggaaaagcgagcatgcggagagagcctcaaacacaaaaaatggcctagtcttgtaatgagtctagccaaatcatgtaagctccgactttcaagagagatcaacagaaaacttcgtcaatccggataaatcaagaaaattatgataatggaaaggaggctggacattctactgccgacgcaacccctggttttggagtcagtgagacaagtggaactaaagaagaatatggatcaaaagagtttatccagttgacacctgatagactcactacatcagttttcagttcaagaacatttcaattcttgctgataaagatagttgccgataaagataggcaaactgttacctaccaatcaaaggaggttgtttcaattgagttagaggtatcaaaggaggagccagtatatatagagcaagttttgatgaagggagttgcctctatttgagaccaccaggtactcaagtgcttcccgtagttcctaggcattttatgatggatatgatagagaaatgtcttattgacaagaatatactagggctacagggataatagggttgggaaggtgaggacttctttggttgctgtcaggaacttggaaacaaagggagaaaggggttggaatcaaaggttttgatttcgtttttgatttataaggaaataatgggtagtggatggagtcgaggataggaaagaggtttaccagttgcaccattgaatatgtaattagagacactatcctcttgttagggaacacgactatcacaagcacgtaagggtgagtgaaagctccgacatggacgtggtttattcgggtatgttggcacgaagccttcgtgtctaggtttggtgttgggttaagtgcaactccttaggaaggcaaataaacttgggacagatttgatagttgtcggaagttgcacaatgatgatattttctttatccaaacgctacgaatgattgcacatatagtaactagagttatttctcatttgagcttttatatgtaagaatcaaataaaatgattgatgaaatgcatgaaagctcaaatgagaaataactagttgtgagaatgcacgggggaaaaatatattatattgattaaagtgttgtacaaccctatttagatacagtaattacataataataggtatctacttcccgatgtgggacactagacatgactaactacttaacaatccccctcaagccggtgcatataaatcatatgtatcgagcttgttacagatgtaactaatacgagaaccagtaagagacttagtgaaaatatctgctagctaatcattcgactttacaaactttgtaacaatatctcttgagagtattttttctctaacaaagtgacagtcgatctcaatgtgtttagtcctttcatagaacaccggatttgacgcaatatgaagagcagcttgattatcacacaccagttccatcttgctgatttctccgaacttcaactccttgagcaactgcttgatccaaactagaatcacacgttgccacaaccatggcccgatattcggcttcggcgctagatcgagcaactacattctgtttcttgctcttccaagagactaaattacctcctactagaacacaatatccagacgtagaacgtcaatcagcaggtaatcctgcccaatcagcatctgtgtacccaacaatctgctcgtggcctcgatcctcaaatcgtaaccctttgcctggagctgactttatataccgaagaatgcgaacaactgcatcccagtgactatcacagggagaaaccataaactaacttgcaacactcaccggaaaagaaatattaggtctagtcactgtgtggtaatttaatttgccaaccaacctcctctatctcgtaggatctctaagatgctccccctgtccatgcagaagcttagcattcggatccatagaagtgtcaactggtctacaacccatcattccagtctcctcaagaatgtctaaggcatatttccgctgtgaaataacaatacctgagctagactgagcgacctcaatacctagaaaatacttcaatctgcccagatccttagtctggaagtgctgaaagagatgctgcttcagattagtaataccatcttgatcattgccaataataataatatcatcaacataccactcaactttggcatttctatctcaatttggctggaatatcctggacaatgcccaataacactgcgtctcttctcagtagctggaacaatggaggggcaaatattaaacagaagaaatggtggaaagtagttcctgcttgtatctggtgggtcatgtggaaggaaaagaatgcagagtttttgaagataggcctagctcttagcctcttaccagaaaattaagcttaattgttttttgttatttcatttttggtgcaaagagagctatagggaggatgtacattctttactagatttgctagaagaaatgtaatcgattagaataggcaaggcagttgcagatcttttggggtctgattgtggcttacactatctcctgtaaatatttttaatcttttatataatttgttaccattctaaaaaaaaacataaaccaccagataaatatacagattaggagcagaatgtcgataaagcacagagtgatccgcttcactacgagtcatgccgaactcctgaataattatgctgaacttaccaaaccaagctcgagggaactgtttcaaaccatatagtgacctgcgcaatcggcatacaagaccactagacttcccttaagcaacaaaaccaggtgattgctccatataaatttcttcctcaagatcaccgtggaggaaagcattcttagtgtctaactgataaagaggtcattgacgtacaacaaccatgaacaagaagagacaaccgatgctactttagccacgggagagagtgtcactataatcaagcccaaaaatctgagtgtatccttttgcaacaagacgagccttaagacgatcaacttggccatccgggctgactttgactgcataaacccaacgataaccaacaatagacttacttgaaggaagaggaacaagcttccaagtgccactcacatgtaaagcagacatctcctcaatcatagtttgtcgccatcctggatgagatagtgcctcacctgtagactttgggatagaaacaattgacaaagatgatataaaagcataatgaggtgatgacagacgatgataacttaaatcgacataatgaggattaagattaagagtggatcatacacctttccgaagtgcaatcggtgtactaggaagagacaagtccgcagtaggagcagggtcaagtgtaggatgtgaatcagttgggcctgatgctgggtgcggacgacgatgatatgtcaagagtggtgttccggtggcggggaatctaggaggagccacactagactccccaacggttggaatgggtaagacttatgtggcggaaggtgaaggaggagctatagtaagctctttaaaggtcggtataggtaagacctcagatatatcaaggtggtcagaagaggtaaagaaaggtttagactcaaaaaatgtgacgtcagatgacataaagtaattacgaaaatcaagtgagtaacaacgatatcccttttgaacacgagaataaccaaggaagacatacttgagagtacgaggagctaacttatctttcctaggggctaaattatgaacgaaacaagagctccccaaaacacgaggaggaacagagtataagggtgactgggaaacaatactgcatacggaatctgattctggatgggagatgaaggcattcgattaaccaaataacaagctgtgagaactgtatcgcctaaaaaacgcaacggaacatgagattcaaagagaagtgtgcgagcagtttcaatgatgtgcctattctttctctctgcaaccccattttgctgaggggtataaggacaagaggtctgatgaataattccttgagaagtcataaagtgctaaaattgagaggataactattctaaggcattatcactgcgaaaagtgcgaatagaaacaccaaattgatttttaatttcatcacaaaaattctggaatatagaaaacaactcagaacgatctttcattaagaaaatccaagtacatcttgaatgatcatcaatgaaactatcaaactaacgaaatcccaaggttgagttgactctactatgaccctatatatcagaatgaactaaagaaaaaacagactatgcatgactctcaatactacgaggaaaggaggctcaggtatgtttcccgagctgacatgactcacactctaatgtagataaactaggcactatcttctgaagcttggatgtcctaaacatctgtgaattaggtccggaggatctgtaactagacatgccttggaggaattgagtgggttaaggtagtaaaggccttctaattcaagtcctgttccaatcgtctgtccgtactgcggtcctgcataataaaagaatcattaataaaatatataccacaatggagggcacaagtcaaacgactaacagatgcaagattaaaaggacaaccagggacataaagaacggaatctagagtgacagagggtaggggattcgcttgtccaactccttttgcttcagtttgagacccgttggctaaagtaacagtggaaagagactgtgaatacgcaatatttgacaaaagtgatttattaccagagatatgatcagaagcggttgagtccacaacccattgtccaagagtactagactgggaaacacaagcaaaagaattaccagcaacaaaagcatcagtctgagcaacagaggctacttgtggagatgtctgcttacttgctcgatactgaaggaacttattatactccccttccgataaagaaaatacccggttacctatagtctcggtctgagcaacataagcatttttgggtggacgaccatgtaaagaatagcacacgtcacgagtgtgtccaagtttatgacaataagagcacttgggtctagatcttccaaaacgacctcctcctcgtctattctccatagtttgagatgcccgattgttcacttactgggatacgagaacagatgagtcaggtctctgtgatgagctcactgggtgacttggtgctgcagcaaggcgaagtaatcgagagaataattcatcaactgtggggacagtcggactagccaaaatctggtcacgtactgaatcaaggtcattagggagtccatcaagtgtaagaactagaaacatcttctgtcgttgctcttgttgctttttaatactagcagaaactggcatcaacgtctcaaattcttccatgattgcctgtacttgtcccctagtaagtagacatatccaattcctgtttcttcaagcttgtcattcgcgatattacatcatagaaacgagatatgtcattagtgtataaattacgagccttttcccaaactaaataacatgtctggaatggacggaacaagggcatcaacttggaatcaatagatcgccacaggatactacataactgagcatcgaccttcttcaaaagtgttttggccttttcatcaccttcgctagccttttttgttaaatgatcttgaactccttgacctttacaacacaactcgacagacgaagcccaagctaagtagtttgaacttctcattaaaggttctgaggtaatcataatagcagaacttccagaactcgtgtttttagacccaaatacatccactcccaaagacattattggattgaaaagagatctagcaaattagcaccaaataaaacaaagaatcaactgtggttgcccaaaaactgccggaaaactactgtagttgccggaaaattttcaaagtgctcggaatcaaaaaataaaaatatgggcaggctcggaatggtagagcgatcagactaacctaaaggagtttttctgaaaaaattgacggaacgggctccatgcgctggtgcgtggagtagatctcgccggagaagactgtctccgatcggcgcgtggcggtgcgtgaggcggcttatgacggaggtgttcgctggggtttggtcgccggaagttgggggaccttgtggtggtgttggtttttgcacaacaccgatggaattggttttgacgaaaaatagccctaaaaggtcaccggaattgaagcacggcgacggctggttttttttttccccggatgttttctcactgccgctctgataccatgtgagaatgcacgggagaaaaatatattatattgattaaagtgttgtacaaccctatttatatacagtaattacataataataggtatctacttcccgatgtgggacactaaacatgactaactacttaacactagtaacctcatggttctcatcctacttcattgaccacttggccacatccttgggtgcctgcactgtagttgtagctgtaatgaagatagttttttttcttttctggatactcttatattgtgacaatttttctctatttgctgttaatggatgaggttatgtgactctccggtggtgagaatgttaatgaacatcaagctcacatgtcatttcattttctgattgatcttgctcttcactctttacgagtttaatgtgttagtccttccaagttctgtccatctatctttctggtgtgcttaacccatgtatattggaccacactttgtattcatgctgattgcaacaaagcctgactgatcctgaactcctcctttatgccttaggtagaaattttgtgtgtttagtgttacatgtttcgcttcaaaggaaaaagggagaaacttaaggtagaatcctgctccttgacctttggatccttgcacattgaagtggacagacatgtttgctttgctttgatgagttgttttagtagtcggtctaaacaactgctgatgtattctgctttattgtaagtgtctataatttttatctttccacaatttgctttcagctctttctgcatgtagagaaaataacagaagcttctatttgatcatgtaatattgactgcgcaagttcagttttaaacaactttggctatgcatatgcaagcaatgacctgaaataaatattattttttatgcagggtctgtatggttttcttcagagatgaaagccttaagtgatgactgtgaacgatttgttagtttccttcccggtcacatttattcaagcaaaaatggtatgcccatacgaagctcatttctgagcttgtgcttcatttatgttgatagttgatcatgtttcctatacgatcagcgtacttttgctatttatttcagatttactttaggaccctgtcggaaacagtcttgaaacccttattgatggtgtaattgttatctcttgatcaaccaaaggagtaattacatgtaattattacaaatttgcaataaaataacttttaggataaccagtggagcttaatgaatcttttaggatatttgggatgctagagtgatgtacttttgataatgtcggttaatataaaatcctctgactttgtactgatgtactggctgagcagattttatattactttctagtccctctgcaaataaaaaaattgtgagactgcaatataacaccattttttaatgcatttacaatgtttaaacttgatgtagcagtgaagaacatgtcgaccttaaacagaggttctatttgtcctagataaaggaacatcagcgtaatgaaacattacaggagagaagctctattgagtttttgttaatctagagggagcccgtaaatagaacaccaattcatctgttatatgacttctttttcattttggaacgttttaaaagtttgacaacattttttgatctccgtacactaaactttttgatgtattaaactaactatttccactactttaatattttcttccttaaacaactcatgttagcatcttaaactgtgtgtgttcaataccctcataaaaaattaaacgagtatttttttatatttgcttatgcccttggagattgggatggggaagttcatcatttgaggtgaaaggtaaattcttttggatggacaaaaagtgaacctcgtctttggcatggagggactatttaaatcgtcatcattaccaaagtcatcctttcaaatgtttactttcaagaactattcatgctatttctcaagtatattatgggtgcaggaggactcagaagatggtacaacccaccatggtactcagaaaccattccttctactccatatgatcaccttgtcttacggaaagcttttgagaaggtcattctattttggatgtcgcttgtttctgagttgtacataatatttaggtgccactttgttatattttgaacttcatcaaaagcctttggttttttgaggacacatatccccttgactgactgggcgctgaatttccttgatgtattgtgcttattttgattgtcctcttctttgtaatactcttgcctataaataaaccttctttatcaaaagaaaatgataaaatgttaataacactttgtgatatatgttgaaggggagtcttggcataactggtaaagttgctgccatgtgaccaggaggtcacgggttcaagccgtggaaacagcctcttgcagaaatgtagggtaaggctgcatacaatcgacccttgtggtccgacccttccccggaccccgcgcataacgggagcttagtgcaccgggctgtcctttttttttgcatagactttacatgatattttatttcaatctttatcaattcttttttaccttcacatgcaaattatactaccgtatgtgaaatatgcaatagtttttcccgcaattttcatctttcatgtacctctctctactatccttgtattactactgatttggtgcattagatgttaattttattcccaacctttactttatgcaggctgtagtcaagcgacttatgacggatgtaccatttggtgtgcttctctcaggtggactagattcttcacttgttgctgcagtggccaaccgttatttggctgatactgaagctgcgcgacaatggggatcacagttgcataccttttgcgtaggcttgaaggtggtgatgctcccttttgtaaacttgctctgattagggaattgctagctgtatcatcccaattcacatggaagttctagaccattattgctgtttcttttccatatatagggattttctgaaaatagtaaaaaggaaatggaatttctcattattaaagataccaaatgcctttttgggaaatgatcttacagttgaatctgaaatttccttttgacattgtgattaattctgatatgaatttggtccatcctggctttccttctcttgattgtagattttttttctctttttgcaattatatgcctttgtatttcatatctcttattatgctattattttattatgcatttttatggtactaatatatcggctcctgttgctttttttgagccgagattttgtttatttctgctatcacgtcctcctgaaaaagtgctactatcttgtattcatgcgggagtttgaaatttgcaagtgtataactttacaaaatgattcgaactgatcacagttcattgctaataaacttttataaaaagcaggtattgttgtgatataatgtgacacttaaataaatttaaacctacatcctttcgaaatctctaatagcttcactaatatttcttgtgctaaattcttccaacacctcttatcgatgccaaatttggcagaccttagtgcaattgaaagtgtttagtgttctttatgcagtaggtatgttattgtccaaaatgacagaaataaagttagagatttgttgaaaagccacttggtgtgattgagcagttcggagatgagtgatttatccatctttttatacttttagtgttttgttttcttttatattgttttctcttttgcttttgtcattgtaattaaggttgtcttttgtttgactttagggttctcctgatctgaaagctgccagagaggtggcagactaccttggaactcgtcaccatgagtttcactttactgtgcaggtaactttcttcataaagacatcctatgctgattttccttataggagtataactgcttaagtcaaattggctatctacttctttctattgctacatcaggaaggaattgatgcactagatgaagtcatttatcatgttgaaacatatgatgtgaccactatcagagccagtacaccaatgtttctcatgtctcggaagataaagtccttgggtgtgaaaatggttctatctggtgaaggttctgatgaaatttttggcggttatttatatttccacaaggcacccaacaantttacacaaaaatgacacaagttatgcagaaaaaatagtcctcaatgtcatgggagaccagggttcaaatctgaggttaaaaaaaatactaggtgaactcttctaatccgtttaagccttggtagatagagttaactagtatatgagctagttagagctagcaggtacctggtagattagtgcaggtgcacacgagctgactcaaaaccaccattattaaaaaataagaaagttttcaatgttgttccaccgtgaattcatgatgtgccgactttcctgtgtttatctctggatagatgaagagtgtttttggatcttgattaattctgtttggcccctttgaggttctgcaagctatttctagactcaaacttgctgcgatctatgttaggtctagagaatatctgccaaataaaacaatggaaggtacactcaagtattttatctccatattacaagtcagtgttagttgaatgggtctgatatatgggacagaaaatggcttcatacccataacctcattaaaatgttgctgatgtgctgatctcatctgtacatctagtataatcctaattacaaattaatgcatctctttgcggtgactatagtatgctgaagaacttttcttgaaacattgcagatcagacctgatctcggaagaatagaaaagtgggttctacgcaatgcttttgacgatgatcagaatccttatctgccaaaggtttgtttgttttcttgtatcaggtccaaaatcaaaatctttgtttattcatttgcataaacaggcagtagactcccaatacattgtgtacacttatgcacaaatgtatgagatgtgtattatatgtgtcacatataagggtatttccacatggtgtttattgatctagagaaagcgtacgacagggttcctagggaggtcctatggagatgcctagaggttaaaggggtcccggttgactgcattagggtgattaaagacatgtatgatggagctaagactcgaattaggacagtaggaggcaactccgaccattttccggttgttacggggttgcatcaagggtctgcgttcaaccctttcctatttgccttggtgatggatgctataaccgcatcatattcaaggggaggtgccatggtgcatgttatttgctgatgacatagtcctaattgacgagacacgacgcggcgtcaacgagaggctagaggtttggagacatgcccttgagtctaaaggtttcaggctgagcaggacgaagacggaatatctcgagtgcaannnnnnnnnnnnnnnnnnnnnnnnnnnnnnnnnnnnnnnnnnnnnnnnnnnnnnnnnnnnnnnnnnnnnnnnnnnnnnnnnnnnnnnnnnnnnnnnnnnnnnnnnnnnatcgtatatgggtagggtggatgaagtggaggttagcaacgggagtcttgtgtgacaagaaagtgtcaccgttactaantctcgagtgcaactttggggccgagccgatggaagcatgagtggaagtgaggctcgactcacaagtcatccctaagaggggtagtttcaagtaccttgggtcagttattcaggggaccggggagatcgacgaggatgtcacacatcgtataggggtggggtggatgaagtggnnnnnnnnnnnnnnnnnnnnnnnnnnnnnnnnnnnnnnnnnnnnnnnnnnnnnnnnnnnnnnnnnnnnnnnnnataggggtagggtggatgaagtggaggttagcaacgggagtcttgtgtgacaagaaagtgtcaccgttactaaaaggtaagttttacagagcagtggttaggcctgctatgttgcatgggaccgagtgttggccggttaaaaattcacacatctagaagatgaaagtagcagagatgaggatgctgaggtggatgtgcgggcatacaaggatggacaagattaggaatgaagttattcgagagaaggtnttgagccgagggtctcctggaaacagcctctctgcccctcggggtaggggtaaggtctgcgtacatactaccctccccagaccccattggtgggattatactgggatgttgttgttgttgttgttgttgttgtacatataagggtattatatgtacacactcctcccacctttcacttatatattcacgtaaaacacatgcatgtgtaaaacctatatatgtgtgtgtgatatatataataaaatgatgtttgaaaagacattatgatcaagtagttgatcttcatctgctttccgtttttagcatatcttgtataggcagaaggaacagttcagtgatggagttggctacagttggattgatggtttgaaggatcacgcaagcagactggtgagctttttagttgttttctcttccctcctcttccattctttatcccttcctttgtggttttgttgaacacatctcgtatatttggtccaggtttctgattctatgttagcgaatgcaagtttcgtttacccgcataacacacccacgacaaaggaaggatactactatagaactatttttgagcgatatttccccaaggtgggtcttagatagtcttcttttccttgttattcatgttcaatttttgatattttgtcccaaacaatgttttctttttcttccttctgttaacaaggtcgcttctatcttcatatttgttgataaaggtaatcacattgataactattatttggagcagaatgctgcgagggaaacagttccaggtggtccaagtgtggcatgcagcactgcaaaagcagtagaatgggacgcagcttggtccaagaatctagatccatctggacgagctgcactcggtgttcatgcagctgcttatgaggatgcatcagaggttaaaaccacagtcgcaacagatacccctcagaaacttgaagttgataaagctgcagtagctgtttga

SEQ ID NO: 10 - protein, 581 aa, Nicotiana tabacum
MCGILAVFGCIDNSQAKRSRIIELSRRLRHRGPDWSGLHSHDDCYLAHQRLAIVDPTSGDQPLYNEDKTIVVAVNGEIYNHRDLREKLKSHQFRTGSDCEVIAHLYEDYGEDFVHMLDGMFSFVLLDTRDKSFIAARDAIGITPLYMGWGLDGSVWFSSEMKALSDDCERFVSFLPGHIYSSKNGGLRRWYNPPWYSETIPSTPYDHLVLRKAFEKAVVKRLMTDVPFGVLLSGGLDSSLVAAVANRYLADTEAARQWGSQLHTFCVGLKGSPDLKAAREVADYLGTRHHEFHFTVQEGIDALDEVIYHVETYDVTTIRASTPMFLMSRKIKSLGVKMVLSGEGSDEIFGGYLYFHKAPNKEEFHQETCRKIKALHLYDCLRANKSTSAWGVEARVPFLDKEFVNVAMNMDPESKMIRPDLGRIEKWVLRNAFDDDQNPYLPKHILYRQKEQFSDGVGYSWIDGLKDHASRLVSDSMLANASFVYPHNTPTTKEGYYYRTIFERYFPKNAARETVPGGPSVACSTAKAVEWDAAWSKNLDPSGRAALGVHAAAYEDASEVKTTVATDTPQKLEVDKAAVAV

SEQ ID NO: 11 - DNA, 17971 bp, Nicotiana tabacum
  misc_feature (1389)..(1389): n is a, c, g, or t
atgtgtggaatactagcagttttcggttgcattgataattctcaggccaagcgttcccgaatcatcgaactttctagaaggtagaatttttttaaaaaaaaaattgcattccaatttttctacagcattcttattctttggggtgacaatggtatgcatgtgttttggatttgctattcgtggacttgttcgctttctcgtggtcttcgatttgtttttgttaatttataatcagtgtttttatatggatttcttttttgaatctctcaaatatatgacatttgatttccacgagaaaatttggcatttttatggttcttatgatatgcggttaacccttcgccttgcatcgcttcagcgctttaaaagacgaaatgatggctattagtaatactgctagagtggttattgaattacattaaataacagattgctagtagatcaaattcagaatgacagtgaaatatctctggaaacttgaatccccgttcaattcgctggtaaaacctggcaaaaaaatagctttatctcaaaggagagtatgtcactgtgaaattggtggtatgtgttgtttaagctttaaggcatgatatgctgctcttaggtgatgtcaggatgataataccatccttttcacactagactcagctttgaagcactttcatctcagttaatcggtggaggaaaatctagtttgctttgggcataatataccaaatgtcttccttttgttttctagtgttgtttctcaagaattgaaaaaccaacctacaatatagtgatataattaactagttagctcttcctgtttttctgaaaatttccaataattgagaagcgtttacaggtcaattagtaaagggagaacggaacatttttttcctctaaagaacttctctttttccatacagaatgactttctatacaaggcctaagtctgctttagtgtctgcgattaagcatcttctgggaaacttcacacttgaaagaagtagaactaggagggggcaggtctagcaagataattgcttcagtcatttctcataaaaaaacattgtttcattcattatgtgcattcatatagagttggttaagctgctaagctgagctaatagtatgatagctatgaatctcgacaaagtaggttgcttcttagggctttattctttggctccgtaaagaatttcttttggaagggcttcagagtgggtaggactgttctgatgataagctgtaacaccaacgaaacaagcctttgtagctgtggaagtccgagggggtggtggtggtggtggtggtgtgagagttagagtggtggaggagaggggaggagtgaagagaagtttatattttaaagaatagggccttgagaacttttagtagtgagcngggggggggggggggcagaggggaggagtgaagagaagtatatattttaaagaatagggccttgagaacttatagtagtaagcatgcattattattattgttgttattattattattattattatttttattattatgtaagatgtaattacttagctaatgaggtttttccaactatttccaaattgtgaaatgtgttgaaagcataattaagtatataaaagcgtgttctttctaatatctttagctttaagaggagataatcacaaaatttatcttgataatatagcagacaatttttcctagttcaaatctcacgtcacccttcataaaaaatttccacgtgcttggcttgcatgttaggggacgtcttgacataattaaacaaatataattgtccctctctaacagcttaagcttttagatgaggcggtcaacaattcaacaatttgcatttgtttgataagaagttatattaaaagaacacttaaaaggtgtcagtatgtgcacaaactcaaggtgtagactaactagaagtcaattcaaattttctgcttgttctctctgttttacttcttttgcactatagaaattgcatttccagcattcccgaaagctgcttcctttgcatatagacatcacatttccagcgtgtctgataagcgttcttgcttattcctgtccctctacttggttgattttcctctcacttagttcactgtcttcttgcacgcattatcaaattgtgttctcaattctcttgccttcttttcatctgaccccacaaaatacctcccaaaaagcctttagtttctgcttttccgagtctgaaattatctgcttattactgcctttcaagtattctgatacgttgaccattgttttccccagtagtaatgcattgttctctgtccaatctctatttttttttttgtgaaccactattctttgttgcttctgtttcgtcatcctcagttccccatcttctcaatttgattttcctcatttaaaaagcgtgtgccccttttcttgtgctaccctctcaaaaatcagttgctgtcatctcgtttgatctgtcatgaacccagttgatgccacatgtttagttctttacctctggacaacttttacttcctgagaaccacaatttcctttccttaagaaattcttagaaattggttatgtaaactgtaaagggaaaatttcccagcaatcaccatttggcctctacgtggcttgcttttcaacttaccgacacgtgttcatccccttttaacaaatgctgaccattatcttctgcttgttggggcatgcttcttacccatggtgttaaccctgatctttcgtatcacatttttcaactcttaattctcatcttataaagtgcatatccttgcctctttagttgatcttgggttgggctgttaatccaaattccatgggctttgctttgaagtatgataagcattagctttactacagtagcatattctacgttgctacagacatgaaattttcctgatttgtctttgatgtgatgtctggcaagtgtagattacgccacagaggacctgactggagtggattgcatagccatgatgactgttatcttgctcatcaacggttggcaatagtagacccaacttctggagatcagccactttacaatgaggacaagaccattgttgtcgcggtagggaaatatttattatatcatttcttagatagttaagtattttaccagtacatggactttggacaatatttgtgcgttttgatcttctatagcacaaacttttctcgtaggataaatttcctctactttgagtgaatcttaacaggaaaatcggaataaacaatttgtgatttcgaaatttttagttcttacatatttgaaacatgtgcggtgaagtaactaggcgcttgactaggtgaatacggagaatttcctctactgttatcgatattttctcagttcatttgaaagatctctgggtcgtctagcagtacaactatttaggcaacttaatcaaatccccttcccatgagtttcactttcttgacttgttttatattttgacattttgcaatgccgaaaataaattgtttttccattttatgacctttaaaatgttgaggtgaagggctaggcggtactttaatcgacttatcggcaacaatgtattagatacagagcacaaacttgtttgggtgcctaaattgatatttttgaaaagtcgatggagtaaatggaaatatggattagcaaaaatattgaaatagtagatctaaacaatggatgactgaatttagaggaggaccttttcttctttccttgttgaagtggttataagagaattattggaagaaaatgtaagctttagggtagtgttgcaccataacagtcatgctttccctcaattattagtgtagctgatgaatgcttttggaaaggtggctgattttttgctgcgtattttatgtctttcatcatctcaaaatttgttgtgttttaacagtgcttggaaggcctagagtcttctgaaaaaagtaggctgagaaaacatgagtaagcaaatttcttcctgctggcaattaatctttgtatatgaggtgaagccacataatctaacatggtattagacatataaatattatttttgacatagagcagacagaaatcttgggtctagttgctatctcccttcctaataagatgccctcattgctatatcccaaaacagattcaccctagaacgaataaatctctccttgcagccacatatatattaataagtagtgtaacactaaaacatttgtgcttctgcaaagtctgttgaagtgggcgattaagtaataaattgtgtgagtttgactgaagagaaagtaataaattgtgtgagcttctcacattttcatgataatgtcaattcatctgattgaactttttgaaggacatctccttttctaaaagtttttgttcacttcctgaaaatggttgctttcccaaatgtattctcctgtattttccttgtgctttatgttgaccaggatgactctggccttccctttttcaaatggtgacttcattaccttttaacaaaagatcaaatagcctttgtatgcttgaaatcgaagcagaatttagggctcaatttctctaggagatgtgtagcagtaacataacacgtggttaaagcaacttttaagcactgccactgtcaaatttgatatgacgctattactatttagagtgtcaaatagtatttcttttgactaccaatttttcaatatcttttttataccttttttctttgactgtgacttatagtatattttatgtagtttcagaatatatattttagtttttaaagaattgatgtctgaaagtacagccaattagatggtttcacccttgtacttcaaatcttataagttgtttaggttaaaggaataatatgcatgattacattgtttggattgaaattcagaagatcaaatgtgcaggcaaaaagcttgcggaagatataattctgtcattttgttgtttagattaacttcccctgtcaaatagctaaaactaattcatactttctcaggatccttcttgattggactactctgatcttcttccatatattgatatatcatattccttttgcttttaggttaacggggagatatataaccatagagaattacgggaaaagctgaagtcccaccagtttcgaactggcagtgactgtgaagttattgcacatcttgtaagtactttcagaatatattcaaataaatatacatgacttctcagtttctgtgcgaagaatgatttcaaaataccatgactcaaatttctcatcaaaagagaaaaaggtggattgtagtaagagaatgagattttttgtcataatttctttcttatggtatttgaactccacgatctacctatcgcagtatgaagactttggagaagacttcgttcacatgttggatggaatgttctcctttgtgcttcttaacacccgtgataaaagtttcattgctgctcgggatgcaattggcattacgcccctttatatgggatggggtcttgatggtatgtaatttttccatttcataatttttggtatattgcccttttaataaatagcctgtgagttatgtgaagttcctttgttgtttccttgttttttatttgcctgatgcatctttgttgttttgcctactataatgctggtttcatgctgttgttacaaacaaatgatgtataatagtgaacagtacatgttttcttgccgctgtagatcaacaatgtaccaagaacatctgtcttaagctagttcaacctaatcttcagttatctatcattccagcgaataacacatgtagagttaaccggacattacctaaggccagctatacaacattgtgaggtgtgactaaggaactctgaacactgtttggagaaatggaaagcaacatatccgtgtttgttttgaagtactataaggaggcagcaaccttgctggatttatcacttgacagcaaatgtcaatggttgaggaacattttttatggctggaggagaaacagagaagagaaaaaataattgattttaaaaaacagaggagaaaattttgtgaagtcgtatgttaatttcaatggctggaggtgcaatatttgacttggcaactagcgtgtagaagtttctggttggggttgagcatggaagacactgttgcttttacaactgtcattagagtcggaaacatattgtattcttgagggagcgttgcaatggataaaaaagtcctacctactacttgatatttgggcattcagaactggttgtctaaagctgagaaggaagaaaaggatttaaaatggtgagtattgtaggctttcttttctgtccagggtgcctggactagttccctgaattgggatactggtggaggatttcctgaaattgatcatggccaaagagatatgtcaggggataagaacattgaaggatcaaaggaaggtgctgcgctaagttttgctagaaatgaacagttccactatggcttttgtcaaagatgggaattgaattggccccaacttctgggcatctccatccatcgtcaggtgaacaaaagtaaggttacaatggtagaatttttcattatttcaaacaagtaaggtgaagtcgtcagcaatcattgcctgagaaggaaccaggaacaaaatctagaagatgtctgctaaagtgctaatagataatctgccaaatttagcacggtaaggctagtgcagatctggttcaaattttaaattggtccaaaatgctttaataaatgtcggacctcgttttggtcccccaaaaggttgctatataaagacttgacaaagaaacaggtgaaggagaagcccaaacaattgaacaaactacacctagcctaaagaaagtggttgatagtttggtcggaggaggaagagcgagcctgcggagagagcctcaaacataaaaaatgacctagtcttgtaatgagtctggccaaatcaagtaagctctgactttcaagagagatcaacagaaaacttcgtcagtctagataaatcaagaaaattatgataatgaaaaggaggctggacattctactgccgaccaaccctggttttggtgtcagtgagacaagtggaactaaagaagaatatggatcaaaagagtttatccggttgacacctgataaactcactacatcagttttcagttcaaaaacatttcaattcttgctgataaagacaggcaaactgtcacctaccaatcaaaggaggttgtttcaattgagttagaggtatcaaaggaggcggcagtatatatggagcaagttttgatgaagggagttgcttctattggagaccaccaggtactcaagtgcttcccgtagttcctaggcattttataattgatatgacagagaaatgtcttattgacaagaatagactaggactacagggataatagtgttgggaaggtgaggacttctttggttgctgtcaggaacttggaaacaaagggagaaaggggttggaatcaaaggttttgatttcatttttgatttatgaggaaataatgggtagtggatggagtcgaggatgggaaagaggtttaccaattgcaccattgaatatgtaattagagacactatcctcttatttgggaacacgactagggtgagggaacgctccgacagggatgtggtttattcgggtatgttggcacgaagcttttgtgtctaggtttggtgttggcttaagtgcaacaccttaggaagacaaacaaacttaggacagatttgatagttgtcggaaattgcacagtgatgatattttcttcttccaaacgttgggaatgattgcacatgtagtaactagagttatttctcatttaagcttttatatgtaagaatcaaataaaataattgatgaaatgcatgaaagcaactgtcttacgcctgaatgcttttaaaaggcatgctttacaaagtttttggtacatctatctgacatgacacactaacattcactcttatatgtgtacatatttaactaagtccaagcctaactatctaactggagatatcaaagttcttagctctttaaagctttcttaactttaggaagatcctgcagtgttgtttttttataaccgtggtatccaggctagcttgcacacatctcgactaattccaccgggtgcttgctatctcccaccaacacagattacctggtaactcatgggaagaaatcacctattgttttgagtctgctggcatttgaagttttggactactaacctcatggttctcatcccacttcattgaccacttggccacatccttgggtgcctgcactgtagctgtaacgaagatagtttttttttccgggatactcttatattgtgataatttttttgtattcgctgttaatggatgaggttatgtgactctccggtggtgagagtgttaatgaacatcaagctcatatgtcatttcattttctgattgatcttgctcttcactctttacgagtttaatgtgttagtccttcccagttttttttaagagcgagaagcgcaaaaaagcgacaagggctcgcctcgcttcaaaagcgaagcgcaaagcgaagcgcacactttattaaagtgaagcgcaattcttaaaaaacataatgtaaaccttgcaaagacacaatataaaattataaataatcaaaaagttcaaattgtcaaaatcaaagctactaaattactagaatcaacctcttattcttctactcttcttgttcttcttcaagattgtcaaaatcttgaattcctctattatcttcatattgctcgtcatcttcctcctccccctcctcttcctcttcatgatcactttcatcttcatcaattagggatagggatcgacttgtagtagccacactttttcccttcctaatcgagcttgaacttgaagtattcccccttaaaccataaggattctccccaactccactagcaaccgcaacatcaccccaagtgaaattagaatcgccttcaaatacttcttcatcttcacaattttcggggactccggttagccactcattagcctcatcaatattgtccaaaagaattggatcaattagattgcggtggttgtagcgacgcctcaatgctctattgtattttatgaacactagattatggaggcgcttcaaggttagtcgattcctcttctttgtatgaatctgcaaacaagatgtgtcaactaattagtaggagttgggacaattgagatataatttactttatctcaaaacacgaaataattctttttatttctcacgtgttcaaaaacgctccagttcctttcacatccggatgagctacaagttaaacttagaactctgatggcgaaagtctgtaaattcggagtctctacaccatattggtcccaccactcaactatagaagtgaaaaaaaaaaattcaagagttaataagtataaaaaatacattaaagttagagctataaaatatagaagcacttggtcacctggcgatttcgtctttctttgtttaatagcaagtcggagcttaaaaagtccctcagctgccttgtaaatagcaagctgatctactatcttttcttgcatgtcttcatctggggtcaacttgataacaacctcatggaatcctgtccacacttctctagccaatgaattattctcatgctgatcataaaagagtgacgggttcagaataagtccagctgcatgcaaaggtctatgaagttgctcactccatcttgcatcaatgatctgaaagacctttgcatatttctgctcatcagtgaatgatgcttgaatagcctccttggccctatccatagcttcatagaggtagcccattggtggtttttgctccccatccaccaaacggagtactttaaccaaagggccaccaattttaagagcatgaaggacattattccaaaaagaataagaaagaataatgcgtgcaacatctttccctgcactttcctttgcaaatttactcttgctccattcctctgaagtgaacaactttctcaaattggatttttgcaagtggatactatgtaaagtcaagaaagcagtggcgaaccttgtcttgcccggtttcaccaaatttttttgtccggtgaatcttctcatcatattcaataacaagggccgctgagaaatataagaatgtaccctaacgccctggccaaaaactgtagagaagggtttttccttgaaaatgtccccgaagattaagttgatacaatgagccgcacatggagtccaatagacattcttgtacgctccttccaccatgccacccgctttcacattttcactcgcattatcagtgaccacttgaacaactttgcttgggccaatcttttcaatggtgttctgaaacaaggtgaacattttgatgtggtcagtggatgagtcgctagcatcaatggactcaagaaacaaacttcccttgggagaattcaccaacacgttaataatcattttcccagttcttgccgtccacttatccatcataatggagcagccatacttgttccacgcaactttatgttcctccacaattttattagtctcctccacttccttatttagataaggacctctgatttcatgataagtgggaggcttcattccaggtccgtattgaccaacggcctcaataaagtctccaaaagtgtcagtatagttgacacaattgaaggggagcccagcatcatagacccatcgtgcaaaagctctaactgcacgatccctcaaaatgtccttagcaattttttgtacatcttttccaccgctctttccttccggcttctttgggaaatagcaatctataggacctttagtcctactcgtacccgtcgatccatggcttgaagagattgcatctcttccccgttttgttggaagtgacaattcttcaatatcatcatcaccatcatcatcaagattggtcaccaatggttgatgactcatttgatttttttgctccttcttcttctcaacaaaattctttatttcatccctcacctccggtggacatttcggacaacttgtgacgtttctatcgccaccaataagatggaatttaaagcgataaattccacccgttgtaatcttgttacaaaacttgcatacaatatttgtattcttctcattaactctatcgccatatcgccaagccgggtctttatctttcgatctttgagacattttgaaatccctattaagatataagaaaatacataatcaaataaactgaaaatacatataatatatataataattaattttataaaccgaaatacacattaaaaaaatcaaataaactaaaatataacatatataattttctaaattgaaatacatataaaattaatcaaataaactgaaaacataacatatatataataattaattttatatactgaaaaatgcattaagaaaatcaaataaactgaaaaatataacatatataaataataattaattttatatactgaaataaaaatcaaataaactaaaatataacatatatatataataattaattttctaaaatgaaatacatataaaattaatcaaataaactgaaaatataacatatataaataataattaatattatatactgaaatatacattaaaaaatcaaataaactgaaaaatataacatatataaataataattaattttatatgctgaaatatacattaaaaaaatcaaataaactgaaaaatataacatatataaataataattaattttataaactaaaatacatattaaaagtaataaataagaagaataaaggggggaaaaaaacaaaatgggttagagataaaaggaagaagaagacgctgaagtctgaacagtgcaaactggactgtcagagtctcagagataaacgaagaagaagaaggaagaaagaaggaaaaagaaagaaaaaaaagcagaatctgacgggaccaagaagaagaaagaaagaagaaagaaaaaaaagagaagaagaaaattacctggactggtcagcaatgtcaatgaagttgaaccctaggctttggtcgacctcgatcgaagaagagagaagaagaaatggccattttttgtcaatttagggtctgttttgtataatagaaaaacagacccaaagttttttttaaaaaaaaaagggcctgcgcttttttaacaaaagcgatcgcttcgtcgcttcctccgttgaagcgtgcgcttccctcggtcgagtcgcctcaggcagctagaagcgacactgagtcgcgtcgcgtcgcttcgcgctttaagcgcgaagcgatcgcttttctaaacactggtccttccaagttctgtccatctttctggtgtgcttaacccatgtatattggaccacactttgtattcatgctgattgcaacaaagcctgactgatcctgaactcctcctttttgccttgggtagaattatttttgtgtttttagtgttacatatttcaatttaaaggaaaaagggagaagcttaaggtagaatcctgctccttgacctttggatccttacacattgaagtggacagacatgtttgctttgctttgctttgatgagttgttttagtagtcagtctaagcaactgctgatgtattctgctttattgtaagtgtctataatttttatctttccacaatttgctttcagctctttctgcatataagagaaaataacagaagcttctattcgatcatgtaatattgactgcacaagtgcatatttaaacaactttggctatgcgtatgcaagcaataataaatattactttttatgcagggtctgtatggttttcttcagagatgaaagccttaagtgatgactgtgaacgatttgttagtttccttcccggtcatatttattcaagcaaaaatggtatgcccatacgaagctcatttctgagcttgcgcttcatttatgatcagcgtacttttcctatttatttcagatttactttaggaccctgttggaaacagtcttgaacccttattgatggtgtaattattatctcttgatcaaccaaaggagtaattacatgtaattattacaaatttgcaacaaaatcttttaggataatcagtggagcttcatgaatcttttaggatagttgggatgctagagtgatgtacttttgataatgtcggttaacataaatcctctgactttgtactgatgtactggctgagcagattttatattactttctaatccctctacaaataaaaaaattgtgagactgcaatataacaccatttttttaatgcatttacaatgtttaaacttgatttagcaacgtagaacatgtcgaccttaaacagaggttctatttgtcctagataaaggaagatcagcataatgaaacattacaggagaggagctctattgagtttttgttaatctagagggagcccgtaaatagtacaccaattcatctcttatatgacttctttttcattttggaacgttttaaaagtttgactacattttttgatctccgtacactaaactttttgatgtattaaactaactatttccactactttaatattttcttccttaaacaactcctgttagcatcttaaactctgtgtgttcaataccctcatataaaattatacgagtattttttttatatttgcttatgtccttggagtttgggatggggaagctcatcatttgaggcgaaaggtaaattcttttgaatggacaaaaagtgaacctcggtctttggcatggagggactatttaagtcgccatcattaccaaagtcatcctttcaagtgtttgctttcaagaactattcatgctatgtctcaagtatattatgtgtgcaggaggactcagaagatggtacaacccaccatggtactcagaaaccattccttctactccatatgatcaccttgtcttacggaaagcttttgagaaggtcattctattttggaagtcgcttgtttctgagttgtatataatatttaggtgccactttgttatattttaaacttcatcaaaagcctttggattctttgaggacacatatccccttgactgactgggagctgaatttccttgatgtatagtgcttattttgattgtcctctcctttgtaatactcttgcctataaataaaccttccttatcaaaagaaaatgataaaatgttaaaaatactttgtgatagatgttgactatagactttaaatgatattttatctcaatctttatcaattcttttttaccttcacatgcaaattatactacagtatgtgaaatatgcaatagtttgtcctgcaattttcatctttcatgtacctctctctactatccgtgtattactactgatttgatgcattaaatgctaattttattcccaacctttactttatgcaggctgtagtcaagcgacttatgacggatgtaccatttggtgtgcttctctcaggcggactagattcttcacttgttgctgcagtggccaaccgctatttggctgatactgaagctgcgcgacaatggggatcacagttgcataccttttgcgtaggcttgaaggtggtgatgctcctttttgtaaacttgctctgatttgggaattgctagctgtatcatcccaatttacatggaagttctagaccattattgctgtttcttttccatatatagggattttctgaaaatagtaaaaaggaaatggaatttctctttattaaagataccgaatgcctttttgggaaatgatcttacagttctgaatcgaaaatttccttttgacattgtgattaattctgatatgaatttggtccatcctggctttccttctcttgattgtagattttccttctcttgttacaattatatgcctgtctttttgtcttactctctgagacaggcaatgtaactccagttgcaaggtttggtaatattgacttgtttatttctgttatcacatcctcctgaaaaagtgctactagcttgtattcatgcgggaatttgaaattttcaagtgtatagctttacaaaatgatcagaactgatcacagtcattgctctaaataaaattttctaaaaagcaggtattgttgtgatataatgtgacacttaaataaatttaaacctacatcctttcgaaatctgtaatagctccactaatatttcttgtgctaaactattccaacacctcttatcgatgccaattttgacagaccttagtgcacttaaaagtgtttagtgttctttatgcagtaggtatgttattgtccaaaatgacagaaataaagttagagatttgttgaaagccacttggtgtgattgagcagttcggagatgagtgatttatccattttatatacttgtagtgttttgttttcttttgcttttgtcattgtaattaaggttgtcttttgtttgacattagggttctcctgatctgaaagctgccagagaggtggcagactaccttggaacccgtcaccatgagtttcactttacagtgcaggtaactttccacaaagacatcctaccatgtgaccaggaggtcacgggtttgagctgtggaaacaaccttttgcagaaatgcagcgtaaggttgcgtacaatagacccttgtggtccggcccttccccgaccccgcacatagcgggagcttagtgcaccgggctgcccatcctaagctgattttccttataggagtataaccgcttaagtcaaattggctatctacttctttctattgctacatcaggaaggaattgatgcactagatgaagtcatttatcatgttgaaacatatgatgtgaccactatcagagccagtacaccaatgtttctcatgtctcggaagataaagtctttgggtgtgaaaatggttctatctggtgaaggttctgatgaaatttttggcggttatttatatttccacaagggacccaacaaagaggagtttcaccaagaaacttgtagaaaggtggatctcattgtcatttcttcagtcattcaggattattggaagtaactgtatttttactagaatacttctttgaactatttctagctctgatggacgctttgatgttaatccagattaaagcacttcatctttatgattgcttgagggccaacaaatctacttcagcttggggtgttgaagctcgtgtacctttcttggataaagaatttatcaatgttgcaatgaacattgatccagagtggaaaatggtaacctacagtgcttccgtctcatttctccaccccccacccccccaaaaaaaagaacagaaaagaattgaaaagagagattcttttcttccttcaaggaagaagggggtaacaaaagaatagctgcaagttatgcagaaaaaatagtcttccatgtcatgggagaccagggttcaaatctgattgttaaaaaaaacactaggtgaactcttctaatctgtttaagccttggtggacatagttaactagtatatgagctagttagagctgactcgaaaccaccattattcaaaaaattaagaaagtcttcaatgttgttccaccgtgaattcatgatgtgtcgactttcatgtgtttatctctggatagatgaagagtttttttggatcttgattaattctgtttggcccctttgaggttctgcacgctatttctagactcaaacttgctgcgacctatgttaggtctagagaatatctgcctaataaaacaatggaagttacattcaagtattttacctccatattacaagtcagtgttagttaaatgggtctgatatatgggatagaaaatggcttcatacccataacctcgttaaaatgttgctgatgtgctgatctcatctgtacatctagtataatcctaattacaaattaatgcatctctttgcggtgactatagtatgctgaagaacctgtcttgaaacattgcagatcagacctgatctcggaagaatagaaaagtgggttctacgcaatgcttttgacgatgatcagaatccttatctgccaaaggtttgtttgttttcttgtatcaggtccaataatcataatctttgtttattcatttgcataaaaggcagtagactcccaatacattgtgtacgcttatgcacaaatgtatgagatgtgtattatatgtgtcacatataagggtattatatgtacacactcctcccaccttccacatatattatgtgtgtgtgtgtgtgtgtataatgaaatgatgtttgaaaagacattatgatcaagtagttgatcctcatctgctttctgtttttagcatatcttgtataggcagaaggaacagttcagtgatggagttggctacagttggattgatggcttgaaggatcacgcaagcagtctggtgagctctttagttgttttctcttccctcctcttccattctttatcccttccttttgtggttttgttgaacacatctcatatacttggtccaggtttctgattctatgttagcgaatgcaagttttgtttacccgcataacacacccacgacaaaggaaggatactattatagaactatttttgagcgatatttccccaaggtgggtcttacatagtcttcttttccttgttattcatgttcagtttatgatattttgtcccaaacaatgttttctttttcttcctttttctgttaacaagatcgcttctatcttcgtatttgttgataaagttaatcacattgttaactattatttggagcagaatgctgcgagggaaacagttccaggtggtccaagtgtggcatgcagcactgcaaaagcagtagaatgggacgcagcttggtccaagaatctagatccatctggtcgagctgcactcggtgttcatgcagctgcttatgaggatgcatcagaggttaaaaccacagtcgcgacagatactgctcagaaacttgacgttgataaagctgcagtagctgtttga

SEQ ID NO: 12 - protein, 581 aa, Nicotiana tabacum; identical to SEQ ID NO: 10

SEQ ID NO: 13 - DNA, 25 bp, Artificial Sequence
  Primer
tcacatatattccctcataacacac

SEQ ID NO: 14 - DNA, 24 bp, Artificial Sequence
  Primer
aagaagcatcccactctacagctt

SEQ ID NO: 15 - DNA, 26 bp, Artificial Sequence
  Primer
atatcttccctcacaacactccaact

SEQ ID NO: 16 - DNA, 22 bp, Artificial Sequence
  Primer
ctaccggaaggatcaaggttgt

SEQ ID NO: 17 - DNA, 330 bp, Nicotiana tabacum
tcacatatattccctcataacacacccattacaaaggaagcatactactataggatgattttcgagcgctttttcccacagaattcagctgggctaaccgttcctggaggagcaagtgtggcgtgtagcacagctaaagctgtagagtgggatgcttcttggtcaaagaaccttgatccttcaggcagggctgctattggtgtacataactcggcttatgagaatcatgtacctgctatggctaatgggaatttgaccaaaaaaatcattggtcgtgtgccttctatggtagaagttggtgctgctcccgagctcacaataaagagttag

SEQ ID NO: 18 - DNA, 364 bp, Nicotiana tabacum
gaccagattggagtgggatatatcaacatggtgatttttacttagcacatcaacgtttagcaattatcgatcctacttctggtgatcagcctctgtttaatcaagataagactattgttgttacagtcaatggagaaatttacaatcatgagaaacttcgtaatcttatgcctaatcacaagttcagaaccggaagtgattgtgatgttattgcacatctttatgaagaatatggagaaaattttgtggacatgttggatggggtgttctcttttgtattgttggatacgcgcgataacagctttcttgctgctcgtgatgcgattggaattactcccctctatattggttggggacttgatgg

SEQ ID NO: 19 - DNA, 1815 bp, Nicotiana tabacum
atgtgcgggatcttggctgttttgggttgttctgatgattctcaggccaaaagggttcgtgttctcgagctctctcgcaggtaggttgaagcatcgtggaccagattggagtgggctgtatcaacatggggactgttacttggcacatcagcgtctagctattgttgatcctgcttccggtgatcaacctctgtttaacgaagataagacgattgttgttacggtaggtaaatggagagatctacaatcacgagcaacttcgtaagcaaatgcctaatcataagttccggactggcagtgactgtgatgtcattgcacacctagtagtatgaagaacatggagaagattttgtggacatgctggatgggatcttcgcttttgtgttattggatactcgagataacagctttcttgttgctcgtgatgccattggaattacttccctttatattggttggggacttgatggtagggtctgtatgaatatcatctgagcttaagggcttgaatgatgactgcgaacattttgaagttttcccaccagggcacttgtactctagcaagaatggcggctttaggaggtggtacaatcctccttggttctctgaggccattccttccactcgttatgatcccttagttctcaggcgtgcctttgaaaatgtaggctgttatcaaaaggttgatgactgatgtcccctttggtgttctcctctccgggggactcgattcatccttggttgcttcgattactgctcgctacttggctggtacaaaggctgccaagcagtggggagcacagcttcattccttctgtgttggccttgaggtagggctcaccggatctcaaggctgcaagagaagttgctgactacttgggaaccgttcaccacgagtttcacttcaccgttcaggtaggatggaattgatgcaattgaagatgttatttaccatattgagacatacgatgtaacgacaatcagagcaagcactcctatgttccttatgtcgcgtaagattaagtcactaggagtgaagatggtcatatctggggaaggatctgatgaagtgtttggtggctacttgtactttcacaaggctcccaacaaggaagagttccacaaggaaacatgtcgcaaggtagattaaagcgcttcaccaatatgactgcttaagagcaaataagtcaacatctgcatggggtttagaagctagagtccctttcctagataaggagttcatcaatgttgccatgagtattgatccagagtggaagttgagattaaaccagagcaaaggaggattgaaaagtgggctctaaggagggcctttgatgatgaggagcatccttatctcccaaaggtagcacatcctgtataggcaaaaagaacaattcagtgatggcgtgggcatagttggatagatggactcaaagcacatgctgaacaacatgtaggtgaccaataggatgatgtttaatgcttcacatatattccctcataacacacccattacaaaggaagcatactactataggatgattttcgagcgctttttcccacaggtagaattcagctgggctaaccgttcctggaggagcaagtgtggcgtgtagcacagctaaagctgtagagtgggatgcttcttggtcaaagaaccttgatccttcaggcagggctgctattggtgtacataactcggcttatgagaatcatgtacctgctatggctaatgggaatttgaccaaaaaaatcattggtcgtgtgccttctatggtagaagttggtgctgctcccgagctcacaataaagagt

SEQ ID NO: 20 - protein, 155 aa, Nicotiana tabacum
MCGILAVLGCSDDSQAKRVRVLELSRRLKHRGPDWSGLYQHGDCYLAHQRLAIVDPASGDQPLFNEDKTIVVTVNGEIYNHEQLRKQMPNHKFRTGSDCDVIAHLYEEHGEDFVDMLDGIFAFVLLDTRDNSFLVARDAIGITSLYIGWGLDGSV

SEQ ID NO: 21 - DNA, 1818 bp, Nicotiana tabacum
atgtgcgggatcttggctgttttgggttgttctgatgattctcaggccaaaagggttcgtgttctcgagctctctcgcaggtaggttgaagcatcgtggaccagattggagtgggctgtatcaacatggggactgttacttggcacatcagcgtctagctattgttgatcctgcttccggtgatcaacctctgtttaacgaagataagacgattgttgttacggtaggtaaatggagagatctacaatcacgagcaacttcgcaagcaaatgcctgatcataagttccggactggaagtgactgtgatgtcattgcacacctagtagtatgaagaacatggagaagattttgtggacatgctggatgggatcttcgcttttgtgttactggatactcgagataacagctttcttgttgctcgtgatgccattggaattacttccctttatattggttggggacttgatggtagggtctgtatgaatatcatctgagcttaagggcttgaatgatgactgcgaacattttgaagttttcccaccaggacacttgtactctagcaagaatggcggctttaggaggtggtacaatcctctttggttctctgaggctattccttccactccttatgatcccttagttctcaggcgcgcctttgaaaatgtaggctgttatcaaaaggttgatgactgatgtcccttttggtgttctgctctccgggggactcgattcatccttggttgcttcgattactgcccgctacttggctggcacaaaggctgccaagcagtggggagcacagcttcattccttctgtgttggccttgaggtagggatcaccggatctcaaggctgcaagagaagttgctgactacttgggaaccgttcaccacgagtttcacttcaccgttcaggtaggatggaattgatgcaattgaagatgttatttaccatattgagacatacgatgtaacgacaatcagagcaagcactcctatgttccttatgtcgcgtaagattaagtcactaggagtgaagatggttatatctggggaaggctctgatgaagtgtttggtggctacttgtactttcacaaggctcccaacaaggaagagttccacaaggaaacatgtcgcaaggtagattaaagcacttcaccaatatgactgtttaagagcaaataagtcaacatctgcatggggcttagaagctagagtgcctttcctagataaggagttcatcaatgttgccatgagtattgatccagagtggaagttggtagattaaaccagagcaaaggaggattgagaagtgggctctaaggagggcctttgatgatgaggagcatccctatctcccaaaggtagcacatcctatacaggcagaaagaacaattcagtgatggcgtaggctatagttggatagatggactcaaagcacatgctgaacaacatgtaggtgaccaataggatgatgcttaatgcttcacatatattccctcataacacaccgattacaaaggaagcatactattataggatgattttcgagcgctttttcccacaggtagaattcagctgggctaaccgttcctggaggagcgagtgtggcgtgtagcacagctaaagctgtagagtgggatgcttcttggtcaaagaaccttgatccttcaggaagggctgctattggtgtacataactcagcttatgagaatcatgaacctgctatggctaatgggaatttggccacaaaaatcattggccgtgcgccgtctatggtagaagttggtgctgctcatgagctcacaataaggagt

SEQ ID NO: 22 - protein, 155 aa, Nicotiana tabacum
MCGILAVLGCSDDSQAKRVRVLELSRRLKHRGPDWSGLYQHGDCYLAHQRLAIVDPASGDQPLFNEDKTIVVTVNGEIYNHEQLRKQMPDHKFRTGSDCDVIAHLYEEHGEDFVDMLDGIFAFVLLDTRDNSFLVARDAIGITSLYIGWGLDGSV

SEQ ID NO: 23 - DNA, 1818 bp, Artificial Sequence
  DNA sequence of ASN5-S stop mutant: ASN5-S_Q66*
  mutation (199)..(201)
atgtgtggaatcttggctttgttgggttgttcagatgattctcaggccaaaagggttcgagttcttgagctctctcgcaggcaggttgaagcatcgtggaccagattggagtgggatatatcaacatggtgatttttacttagcacatcaacgtttagcaattatcgatcctgcttctggtgatcagcctctgtttaattaagataagacgattgttgttacagtaggtcaatggagagatttacaatcatgagaaacttcgtaatcttatgcctaatcacaagttcagaactggaagtgattgtgatgttattgcacatcttgtagtatgaagaatatggagaaaattttgtggacatgttggatggggtgttctcttttgtattgttggatacgcgcgataacagctttcttgctgctcgtgatgcaattggaattactcccctatatattggttggggacttgatggtaggctctgtgtggatttcatctgagctaaaaggattaaatggtgactgtgaacattttgaagttttccctcccggtcacttgtactcgagcaagaatggcgggtttaggagatggtacaatcctcaatggttctctgaggctattccatcaaatccttacgaccccttagttttgagacgtgccttcgaaaatgtaggctgttatcaaacgattgatgaccgatgtcccctttggtgttctgctctccgggggacttgattcgtctttggttgcttctgtcactgctcgctacttggctggaacaaaagctgctaagcaatggggagcacagcttcattccttctgtgttggtctcgaggtagggctcaccagatctcaaggctgcaagagaagttgctgactatttgggaaccgttcaccacgagttcaccttcacagttcaggtaggatggaattgatgctattgaagatgttatttaccatatcgagacatacgatgtaacaacgatcagagcaagcactcctatgttccttatgtcgcgtaagattaaatcactgggagttaagatggtcatatcaggggaaggctcagatgaactgtttggcggctatttgtacttccacaaggctccgaacaaggaagaattccatgtggagacatgtcacaaggtagataaaagcgcttcaccaatacgactgtttgagagcaaataaggcaacatcagcatggggcttagaagctagagtaccatttctggataaagagttcatcaacgttgctatgagtatcgatcctgaatggaagatggtagattaaacacgatcatggtaggatcgagaagtgggttcttaggaaggcttttgatgatgaggagcaaccctatctcccaaaggtagcatattctgtaccggcagaaagaacaattcagtgatggcgtaggctatagttggatcgatggactcaaagcacatgctgaacaacatgtaggtgactgataggatgatgcttaatgctgcacatatcttccctcacaacactccaactacaaaggaagcatactattacaggatgattttcgagaggttcttcccacaggtagaattcagcaaggctaactgttcctggaggaccgagtatagcttgcagcacagctaaagctattgagtgggatgcttcgtggtcgaacaaccttgatccttccggtagggctgcaatcggtgtacataactcggcttatgacgatcatctccccgatgttggtaatgggaatttggacacaacgatcatcgataatgtgccgaggatggtaggagtgggtgctgctgcagagctcacaataaggagc

SEQ ID NO: 24 - protein, 65 aa, Artificial Sequence
  Amino acid sequence of ASN5-S stop mutant: ASN5-S_Q66*
MCGILALLGCSDDSQAKRVRVLELSRRLKHRGPDWSGIYQHGDFYLAHQRLAIIDPASGDQPLFN